European Patent Specification EP 3 485 039 B1, published January 18, 2023. Title: 2 probe signature. Applicant: Imperial Innovations Ltd. The sequence listing filed with the application follows.

SEQUENCE LISTING (40 sequences)

SEQ ID NO: 1 - DNA, 63234 bp, Artificial Sequence
  GENOMIC SEQUENCE FOR IFI44L
gctgccagctgagtttttttgctgctttgagtctcagttttctttctttcctagagtctctgaagccacagatctcttaagaactttctgtctccaaaccgtggctgctcgataaatcagacagaacagttaatcctcaatttaagcctgatctaacccctagaaacagatatagaacaatggaagtgacaacaagattgacatggaatgatgaaaatcatctgcgcaagctgcttggaaatgtttctttgagtcttctctataagtctagtgttcatggaggtagcattgaagatatggttgaaagatgcagccgtcagggatgtactataacaatggcttacattgattacaatatgattgtagcctttatgcttggaaattatattaatttacatgaaagttctacagagccaaatgattccctatggttttcacttcaaaagaaaaatgacaccactgaaatagaaactttactcttaaatacagcaccaaaaattattgatgagcaactggtgtgtcgtttatcgaaaacggatattttcattatatgtcgagataataaaatttatctagataaaatgataacaagaaacttgaaactaaggttttatggccaccgtcagtatttggaatgtgaagtttttcgagttgaaggaattaaggataacctagacgacataaagaggataattaaagccagagagcacagaaataggcttctagcagacatcagagactataggccctatgcagacttggtttcagaaattcgtattcttttggtgggtccagttgggtctggaaagtccagttttttcaattcagtcaagtctatttttcatggccatgtgactggccaagccgtagtggggtctgatatcaccagcataaccgagcggtataggatatattctgttaaagatggaaaaaatggaaaatctctgccatttatgttgtgtgacactatggggctagatggggcagaaggagcaggactgtgcatggatgacattccccacatcttaaaaggttgtatgccagacagatatcagtttaattcccgtaaaccaattacacctgagcattctacttttatcacctctccatctctgaaggacaggattcactgtgtggcttatgtcttagacatcaactctattgacaatctctactctaaaatgttggcaaaagtgaagcaagttcacaaagaagtattaaactgtggtatagcatatgtggccttgcttactaaagtggatgattgcagtgaggttcttcaagacaactttttaaacatgagtagatctatgacttctcaaagccgggtcatgaatgtccataaaatgctaggcattcctatttccaatattttgatggttggaaattatgcttcagatttggaactggaccccatgaaggatattctcatcctctctgcactgaggcagatgctgcgggctgcagatgattttttagaagatttgcctcttgaggaaactggtgcaattgagagagcgttacagccctgcatttgagataagttgccttgattctgacatttggcccagcctgtactggtgtgccgcaatgagagtcaatctctattgacagcctgcttcagattttgcttttgttcgttttgccttctgtccttggaacagtcatatctcaagttcaaaggccaaaacctgagaagcggtgggctaagataggtcctactgcaaaccacccctccatatttccgtaccatttacaattcagtttctgtgacatctttttaaaccactggaggaaaaatgagatattctctaatttattcttctataacactctatatagagctatgtgagtactaatcacattgaataatagttataaaattattgtatagacatctgcttcttaaacagattgtgagttctttgagaaacagcgtggattttacttatctgtgtattcacagagcttagcacagtgcctggtaatgagcaagcatacttgccattacttttccttcccactctctccaacatcacattcactttaaatttttctgtatatagaaaggaaaactagcctgggcaacatgatgaaaccccatctccactgcaaaaaaaaaaaaaaaaaataagaaagaacaaaacaaaccccacaaaaattagctgggtatgatggcacgtgcctgtagtcccagttactcaggatgattgattgagccttggaggtggaggctacagtgagctgagattgtgccactgtactctagccagggagaaagagtgagatcctggctcaaaaaaaccaaataaaacaaaacaaacaaacgaaaaacagaaaggaagactgaaagagaatgaaaagctggggagaggaaataaaaataaagaaggaagagtgtttcatttatatctgaatgaaaatatgaatgactctaagtaattgaattaattaaaatgagccaacttttttttaacaatttacattttatttctatgggaaaaaataaatattcctcttctaacaaacccatgcttgattttcattaattgaattccaaatcatcctagccatgtgtccttccatttaggttactggggcaaatcagtaagaaagttcttatatttatgctccaaataattctgaagtcctcttactagctgtgaaagctagtactattaagaaagaaaacaaaattcccaaaagatagctttcacttttttttttccttaaagacttcctaattctcttctccaaattcttagtcttcttcaaaataatatgctttggttcaatagttatccacattctgacagtctaatttagttttaatcagaattatactcatcttttgggtagtcatagatattaagaaagcaagagtttcttatgtccagttatggaatatttcctaaagcaaggctgcaggtgaagttgtgctcaagtgaatgttcaggagacacaattcagtggaagaaattaagtctttaaaaaagacctaggaataggagaaccatggaaattgaggaggtaggcctacaagtagatattgggaacaaaattagagaggcaaccagaaaaagttattttaggctcaccagagttgttcttattgcacagtaacacaccaatataccaaaacagcaggtattgcagtagagaaagagtttaataattgaatggcagaaaaatgaggaaggttgaggaaacctcaaatctacctccctgctgagtctaagtttaggatttttaagagaaaggcaggtaaggtgctgaaggtctggagctgctgatttgttggggtatagggaatgaaatgaaacatacagagatgaaaactggaagtttttttttgtttgttttgttttttttttgttgttgtttttttttttttttgtttttttgctgagtcaattccttggagggggtcttcagactgactggtgtcagcagacccatgggattccaagatctggaaaactttttagatagaaacttgatgtttcttaacgttacatatattatcttatagaaataactaagggaagttagtgccttgtgaccacatctatgtgacttttaggcagtaagaaactataaggaaaggagctaacagtcatgctgtaagtagctacagggaattggcttaaagggcaagttggttagtacttagctgtgtttttattcaaagtctacattttatgtagtggttaatgtttgctgttcattaggatggtttcacagttaccatacaaatgtagaagcaacaggtccaaaaagtagggcatgattttctccatgtaatccagggagaaaacaagccatgaccattgttggttgggagactgaaggtgattgaaggttcaccatcatcctcaccaacttttgggccataattcacccaaccctttggtggagcctgaaaaaaatctgggcagaatgtaggacttctttattttgtttaaaggggtaacacagagtgcccttatgaaggagttggagatcctgcaaggaagagaaggagtgaaggagagatcaagagagagaaacaatgaggaacatttcatttgacccaacatcctttaggagcataaatgttgacactaagttatcccttttgtgctaaaatggacagtattggcaaaatgataccacaacttcttattctctggctctatattgctttggaaacacttaaacatcaaatggagttaaatacatatttgaaatttaggttaggaaatattggtgaggaggcctcaaaaagggggaaacatcttttgtctgggaggatattttccattttgtggatttccctgatctttttctaccaccctgaggggtggtgggaattatcattttgctacattttagaggtcatccaggatttttgaaactttacattctttacggttaagcaagatgtacagctcagtcaaagacactaaattcttcttagaaaaatagtgctaaggagtatagcagatgacctatatgtgtgttggctgggagaatatcatcttaaagtgagagtgatgttgtggagacagttgaaatgtcaatgctagagcctctgtggtgtgaatgggcacgttaggttgttgcattagaaagtgactgtttctgacagaaatttgtagctttgtgcaaactcacccaccatctacctcaataaaatatagagaaaagaaaaatagagcagtttgagttctatgaggtatgcaggcccagagagacataagtatgttcctttagtcttgcttcctgtgtgccacactgcccctccacaaccatagctgggggcaattgtttaaagtcattttgttcccgactagctgccttgcacattatcttcattttcctggaatttgatacagagagcaatttatagccaattgatagcttatgctgtttcaatgtaaattcgtggtaaataacttaggaactgcctcttctttttctttgaaaacctacttataactgttgctaataagaatgtgtattgttcaggacaacttgtctccatacagttgggttgtaaccctcatgcttggcccaaataaactctctacttatatcagtttttcctacacttcttccttttaggtcaacaataccaagaggggttactgtgctgggtaatgtgtaaacttgtgtcttgtttagaaagataaatttaaagactatcacattgctttttcataaaacaagacaggtctacaattaatttattttgacgcaaattgataggggggccaagtaagccccatatgcttaatgatcagctgatgaataatcatctcctagcaacataactcaatctaatgctaaggtacccacaagatggcaaggctgatcaaagtcgtcatggaatcctgcaaccaaaagccatgggaatttggaagccctcaaatcccattcctaatctgatgagtctatggaccaatttgtggaggacagtagattaaatagatctgatttttgccatcaatgtaaggaggataaaaacttgcataccaattgtacacccttgcaaaatctttctctgatgttggagaaaatgggccagtgagatcatggatatagaagtacagtcaatgttcagctgtaccctcccacaatcccacttccttcctcaacacaattcaaacaaatagactcagactgtttcaggctccaggacaggaagtgcagtgtaggcaaaattgcaaaaattgagggcacaggggtggaggtgggggggttgaataacaagctgtgctaaataattacgtgtaaatatattttttcatttttaaaaattgatttcttttgcacattccatgacaatatatgtcacatttttaaaataaatgcaaagaagcatacatccaaatggaagtgacaacaagattgacatggaatgatgaaaatcatctgcgcaagctgcttggaaatgtttctttgagtcttctctataagtctagtgttcatggaggtagcattgaagatatggttgaaagatgcagccgtcagggatgtactataacaatggcttacattgattacaatatgattgtagcctttatgcttggaaattatattaatttacatgaaagttctacagagccaaatgattccctatggttttcacttcaaaagaaaaatgacaccactgaaatagaaactttactcttaaatacagcaccaaaaattattgatgagcaactggtgtgtcgtttatcgaaaacggatattttcattatatgtcgagataataaaatttatctagataaaatgataacaagaaacttgaaactaaggttttatggccaccgtcagtatttggaatgtgaagtttttcgagttgaaggaattaaggataacctagacgacataaagaggataattaaagccagagagcacagaaataggcttctagcagacatcagagactataggccctatgcagacttggtttcagaaattcgtattcttttggtgggtccagttgggtctggaaagtccagttttttcaattcagtcaagtctatttttcatggccatgtgactggccaagccgtagtggggtctgatatcaccagcataaccgagcggtataggatatattctgttaaagatggaaaaaatggaaaatctctgccatttatgttgtgtgacactatggggctagatggggcagaaggagcaggactgtgcatggatgacattccccacatcttaaaaggttgtatgccagacagatatcagtttaattcccgtaaaccaattacacctgagcattctacttttatcacctctccatctctgaaggacaggattcactgtgtggcttatgtcttagacatcaactctattgacaatctctactctaaaatgttggcaaaagtgaagcaagttcacaaagaagtattaaactgtggtatagcatatgtggccttgcttactaaagtggatgattgcagtgaggttcttcaagacaactttttaaacatgagtagatctatgacttctcaaagccgggtcatgaatgtccataaaatgctaggcattcctatttccaatattttgatggttggaaattatgcttcagatttggaactggaccccatgaaggatattctcatcctctctgcactgaggcagatgctgcgggctgcagatgattttttagaagatttgcctcttgaggaaactggtgcaattgagagagcgttacagccctgcatttgagctgccagctgagtttttttgctgctttgagtctcagttttctttctttcctagagtctctgaagccacagatctcttaagaactttctgtctccaaaccgtggctgctcgataaatcagacagaacagttaatcctcaatttaagcctgatctaacccctagaaacagatatagaacaatggaagtgacaacaagattgacatggaatgatgaaaatcatctgcgcaagctgcttggaaatgtttctttgagtcttctctataagtctagtgttcatggaggtagcattgaagatatggttgaaagatgcagccgtcagggatgtactataacaatggcttacattgattacaatatgattgtagcctttatgcttggaaattatattaatttacatgaaagttctacagagccaaatgattccctatggttttcacttcaaaagaaaaatgacaccactgaaatagaaactttactcttaaatacagcaccaaaaattattgatgagcaactggtgtgtcgtttatcgaaaacggatattttcattatatgtcgagataataaaatttatctagataaaatgataacaagaaacttgaaactaaggttttatggccaccgtcagtatttggaatgtgaagtttttcgagttgaaggaattaaggataacctagacgacataaagaggataattaaagccagagagcacagaaataggcttctagcagacatcagagactataggccctatgcagacttggtttcagaaattcgtattcttttggtgggtccagttgggtctggaaagtccagttttttcaattcagtcaagtctatttttcatggccatgtgactggccaagccgtagtggggtctgatatcaccagcataaccgagcggtataggatatattctgttaaagatggaaaaaatggaaaatctctgccatttatgttgtgtgacactatggggctagatggggcagaaggagcaggactgtgcatggatgacattccccacatcttaaaaggttgtatgccagacagatatcagtttaattcccgtaaaccaattacacctgagcattctacttttatcacctctccatctctgaaggacaggattcactgtgtggcttatgtcttagacatcaactctattgacaatctctactctaaaatgttggcaaaagtgaagcaagttcacaaagaagtattaaactgtggtatagcatatgtggccttgcttactaaagtggatgattgcagtgaggttcttcaagacaactttttaaacatgagtagatctatgacttctcaaagccgggtcatgaatgtccataaaatgctaggcattcctatttccaatattttgatggttggaaattatgcttcagatttggaactggaccccatgaaggatattctcatcctctctgcactgaggcagatgctgcgggctgcagatgattttttagaagatttgcctcttgaggaaactggtgcaattgagagagcgttacagccctgcatttgagataagttgccttgattctgacatttggcccagcctgtactggtgtgccgcaatgagagtcaatctctattgacagcctgcttcagattttgcttttgttcgttttgccttctgtccttggaacagtcatatctcaagttcaaaggccaaaacctgagaagcggtgggctaagataggtcctactgcaaaccacccctccatatttccgtaccatttacaattcagtttctgtgacatctttttaaaccactggaggaaaaatgagatattctctaatttattcttctataacactctatatagagctatgtgagtactaatcacattgaataatagttataaaattattgtatagacatctgcttcttaaacagattgtgagttctttgagaaacagcgtggattttacttatctgtgtattcacagagcttagcacagtgcctggtaatgagcaagcatacttgccattacttttccttcccactctctccaacatcacattcactttaaatttttctgtatatagaaaggaaaactagcctgggcaacatgatgaaaccccatctccactgcaaaaaaaaaaaaaaaaaataagaaagaacaaaacaaaccccacaaaaattagctgggtatgatggcacgtgcctgtagtcccagttactcaggatgattgattgagccttggaggtggaggctacagtgagctgagattgtgccactgtactctagccagggagaaagagtgagatcctggctcaaaaaaaccaaataaaacaaaacaaacaaacgaaaaacagaaaggaagactgaaagagaatgaaaagctggggagaggaaataaaaataaagaaggaagagtgtttcatttatatctgaatgaaaatatgaatgactctaagtaattgaattaattaaaatgagccaacttttttttaacaatttacattttatttctatgggaaaaaataaatattcctcttctaacaaacccatgcttgattttcattaattgaattccaaatcatcctagccatgtgtccttccatttaggttactggggcaaatcagtaagaaagttcttatatttatgctccaaataattctgaagtcctcttactagctgtgaaagctagtactattaagaaagaaaacaaaattcccaaaagatagctttcacttttttttttccttaaagacttcctaattctcttctccaaattcttagtcttcttcaaaataatatgctttggttcaatagttatccacattctgacagtctaatttagttttaatcagaattatactcatcttttgggtagtcatagatattaagaaagcaagagtttcttatgtccagttatggaatatttcctaaagcaaggctgcaggtgaagttgtgctcaagtgaatgttcaggagacacaattcagtggaagaaattaagtctttaaaaaagacctaggaataggagaaccatggaaattgaggaggtaggcctacaagtagatattgggaacaaaattagagaggcaaccagaaaaagttattttaggctcaccagagttgttcttattgcacagtaacacaccaatataccaaaacagcaggtattgcagtagagaaagagtttaataattgaatggcagaaaaatgaggaaggttgaggaaacctcaaatctacctccctgctgagtctaagtttaggatttttaagagaaaggcaggtaaggtgctgaaggtctggagctgctgatttgttggggtatagggaatgaaatgaaacatacagagatgaaaactggaagtttttttttgtttgttttgttttttttttgttgttgtttttttttttttttgtttttttgctgagtcaattccttggagggggtcttcagactgactggtgtcagcagacccatgggattccaagatctggaaaactttttagatagaaacttgatgtttcttaacgttacatatattatcttatagaaataactaagggaagttagtgccttgtgaccacatctatgtgacttttaggcagtaagaaactataaggaaaggagctaacagtcatgctgtaagtagctacagggaattggcttaaagggcaagttggttagtacttagctgtgtttttattcaaagtctacattttatgtagtggttaatgtttgctgttcattaggatggtttcacagttaccatacaaatgtagaagcaacaggtccaaaaagtagggcatgattttctccatgtaatccagggagaaaacaagccatgaccattgttggttgggagactgaaggtgattgaaggttcaccatcatcctcaccaacttttgggccataattcacccaaccctttggtggagcctgaaaaaaatctgggcagaatgtaggacttctttattttgtttaaaggggtaacacagagtgcccttatgaaggagttggagatcctgcaaggaagagaaggagtgaaggagagatcaagagagagaaacaatgaggaacatttcatttgacccaacatcctttaggagcataaatgttgacactaagttatcccttttgtgctaaaatggacagtattggcaaaatgataccacaacttcttattctctggctctatattgctttggaaacacttaaacatcaaatggagttaaatacatatttgaaatttaggttaggaaatattggtgaggaggcctcaaaaagggggaaacatcttttgtctgggaggatattttccattttgtggatttccctgatctttttctaccaccctgaggggtggtgggaattatcattttgctacattttagaggtcatccaggatttttgaaactttacattctttacggttaagcaagatgtacagctcagtcaaagacactaaattcttcttagaaaaatagtgctaaggagtatagcagatgacctatatgtgtgttggctgggagaatatcatcttaaagtgagagtgatgttgtggagacagttgaaatgtcaatgctagagcctctgtggtgtgaatgggcacgttaggttgttgcattagaaagtgactgtttctgacagaaatttgtagctttgtgcaaactcacccaccatctacctcaataaaatatagagaaaagaaaaatagagcagtttgagttctatgaggtatgcaggcccagagagacataagtatgttcctttagtcttgcttcctgtgtgccacactgcccctccacaaccatagctgggggcaattgtttaaagtcattttgttcccgactagctgccttgcacattatcttcattttcctggaatttgatacagagagcaatttatagccaattgatagcttatgctgtttcaatgtaaattcgtggtaaataacttaggaactgcctcttctttttctttgaaaacctacttataactgttgctaataagaatgtgtattgttcaggacaacttgtctccatacagttgggttgtaaccctcatgcttggcccaaataaactctctacttatatcagtttttcctacacttcttccttttaggtcaacaataccaagaggggttactgtgctgggtaatgtgtaaacttgtgtcttgtttagaaagataaatttaaagactatcacattgctttttcataaaacaagacaggtctacaattaatttattttgacgcaaattgataggggggccaagtaagccccatatgcttaatgatcagctgatgaataatcatctcctagcaacataactcaatctaatgctaaggtacccacaagatggcaaggctgatcaaagtcgtcatggaatcctgcaaccaaaagccatgggaatttggaagccctcaaatcccattcctaatctgatgagtctatggaccaatttgtggaggacagtagattaaatagatctgatttttgccatcaatgtaaggaggataaaaacttgcataccaattgtacacccttgcaaaatctttctctgatgttggagaaaatgggccagtgagatcatggatatagaagtacagtcaatgttcagctgtaccctcccacaatcccacttccttcctcaacacaattcaaacaaatagactcagactgtttcaggctccaggacaggaagtgcagtgtaggcaaaattgcaaaaattgagggcacaggggtggaggtgggggggttgaataacaagctgtgctaaataattacgtgtaaatatattttttcatttttaaaaattgatttcttttgcacattccatgacaatatatgtcacatttttaaaataaatgcaaagaagcatacatccaagtaagcgactttttaattgaaacatagtatttgtacgtatttatggggttatgtgtgatattttgatacaagcatacaatgtaatgaccaaatcaggatcattgggaaatccatcacctcaaccatttatcatttctttgtatttggaacattccaaattttctcttctagctatttcaaaatagacaataaattattgttaactatagttaaactgttgtgctatgaacacaagaacttattccttctatgtagctgtatttttgtaaccattaaccaacctcttttcatcatctccttcctctgactttcccaacctctggtaaccaccatgctactctctgcctccatgaaatcaacttttattttaagcttccacgtgtgagtgagaacatcacaggtaagtgacttcttgccatccaattttgctagctgtgtgtgaagaaaaaagcttgctttctttttttctaaaaaggagtttcagagtggaattgctgctaatactttgctctttcatttgtcttttattttaatgaaaatttcacacacagataactagagagtataaatgaaccatactgtaatctgatatagttttatccaattttaaaaatgatttgctttttaaattagaatagttttcttttacttaaatacaaaagcattacaaataaagttgaagaaatctatgactctctactatatattgttttcttatgagatggagtctcactctattgcccaggctggagagcagtgtctcgatgtcggctcactgcaacctcagcctcctgggttcaagggattcttgtgcctcagcctcccaagtacctgggattacaggcgtgcaccagcatgcctggctaatttttgtatttttagtagagacgaggtttcaccatgttggccaggctggtcttgaactcctgaccgcaagtgatctgccagcctcagcctcccaaagtgctgggattacaggtgtgagccaccacacctagcctctcctatattctttacctttctttttatttccagaaggcaacattatctagactttggtataaattattgtcataattgtttttatggttttctgtatgtgtgtatatatttatctaaatatgatctctagtataatttgttaaaattacttctgtttttatataccagcaaaaatggttttacacaataacttaaaaaattaatatacttatattaattttatttttattgatacataatacattacatatttatggggtacaggtgatatttggtgatgcacttagaatgtgtaatgatcaagtcagggtatttgtggtttccatcgctttgagtatttattatttccatgtgctgggaacaacccaagtcttctagctactttgaaatagacaatacattgcttttggccatagtcactctactttgttgttgactaatagaacttctaccttctatttaactgtatatttgtactcattaacctacatctcttcatctctccctcctagacacccacccacccttcctagcctccagtatttatcattatactatccacatttataagatcaacatttttagctgatctaaaatgatgagtgagaacgtgtgatatttcctgtgcctaggttatttcacttaatattctccagttccgtccatgttgctgcaaatgacatgattttactgtttttatagctaaatagtattccattgtgtaatataccacattttctttatccatccacttatggacagttaggttgattccatatcttttctattgttaatagaaattcacaatagaaaggttgctgtgataaacctgagagacaccagaaggaattttaacatattgaccatactaaacaatatttaacatattgattgtattcagctatcttttacaatgtggtgtacagactctaaaatagctcctaattgtccctgtcctattttttttttaatactcatgtccgtgtataatccccccttgtctgtggatggaaactgtgacttaacggtaacaaatagaatttggcaaatgtgatatgttaagattataatgtctgctatgctaggagattctctcccttgctggtttcaatgaagtaagtggtcatgttggggaggcccatttggcaaagaactaagggtgacttcaggccaatgactaactgagaactgaggataacctctgatcattagctagcaagaaatggagttctcatatctacaaccataaggaactgaattctgctaacaaccataggagcttggaagcatgtccttctcccgttaaacattcagaagagtctgcagctgtggctcgcactttgataactgcctcatgaaaaattctgaagcagagaaccaaactggatttctgacccagagaaactgtgagactataaatgtgtgttgttttaagtctctaaacgtatgagaaattgctatgcagcaatagataaatagcacactaaattagttaatactattactttatcggtagatgctttaaggttttccacatataagataatatcatctgtgagcagagatgattatacttcctttataattcaggtaccttttcctttttcactttcttttttattttggcctacttgttctggctaggacattcagtattatgttgaatagaagtggtaaaagtggataatcttgtcttgtactttatcttagaggaaaagctgtcagtttttcactgctgaatatgatgttaactatgaactttttatacatgtatttactatgttgaggtaatttccttctactcctggtttaagtgttttttgttttttttttttttttttttttttttttttaaatcatggaaggacttgggttttatcaaatgtcttttctgtatctattgagatgaccaatttgtattagtcagcgttcttcagagaaactgaaccaacataaaaaaaataaaattaaaaaaaaactaaggaaatttgttatgggaggtggctcatgtggtgttggagggcgagaagtctcactatctgccacctgccagatgtaaagccaggaaagctggtggtgtaattcagtctgaatccaaatgcctgagaactggtggagccagtggtggaactcccagtctgaaatcaaagtcctgggaactgtgggaactgagagagctggaggtgtaagtcccagaatccgaatgtttgagaaccaggagctcagatatctgagagcagaagaagatggatactccagctcaagaatagagaatttgctcttcctctgcctttttgctctatttgggccctcaatggattggatgatgtcagctcatgttggatcttttttatgcagtttactaattcaaatgctaatctaaaatgtgtttgtatattcatttgcctcaacatttcttttcttttctttttttcctttcttttctttttttgagatggagtgtctctctgtcacccaggctggagtgcagtggtgcaatctctgcctcccaggttcaagcgattctcctacttcagccttctgagtagctgggactacaggtgcacaccaccacacccaatttttgtatttttgtatttttgttagagacggggcttttccgtattggccaggctggtctcagactcatgacctcaagtgttccgccgaactcggcctcccaaagtactgggtttacaggtgtgagtcaccacgcctggcctcaagatatttttaaaattcccttttgatttcattttgatccactgcttattccagagggtgtagtttaattctcacatccttgttaattttctagattttctgatattgatttctagtttcattacatggttatgaggaaagacttgatatggtttcaatcttcttagatttgttaagacttgttttttgacctaacatgtaatctatcctggagaacgctcctataatacacttgagaagaatgtgtattttgttgttgctgggtggaatgccctgtatatgcctattaggtccattgggactatagtgttcaagttttctgttttcctattgatcttctgtttggatattttataatggataaagtattgaaagtgggctatcaaaatctccttctcttattgtgttgctgtttctcccttcaattctttcagtgtttgcttcatttatttaggtgctctgatgttggatgaacatatatttataacggttatatttttctggagaattgacccttttcttattatatgatgtccttcatagcctgttatgacaggttttgatttaatgtctattttgtgtgggataaggacacacaccccttgcgggttatcttgcggttcttgcagttaccatttgcaaaggtacccttattatcacttgattttcatcctatgtgtgttcttaagtctaagtgagttcttggggacagcatgctgttgtattttgtcatgacatgctttgactcagtattatccttctttctttccttccttttttttttttggtttgctaatattttgctgaggatcattccatctatatttataaaagagattggcctgtaatttttcttgcttataacgccattaacaggttttggtatctaagttattctctggaagaacatgtgtaagattgtgtattatttattcttcaaaatttggtagaattcagcagctagactctgatccttgagttttcttggggaagtcttaaattaattatgaatttagtttttaaaaatagctatgagatagtcaaattttgtatttacttttatgtcagctttggtaagttgtatttttctagaaatttgtccacttattctcaaatttaattttacaaagttgtttatcttcagaccattttatcgtttatcatttattgcatctggactgatgttttctcttacgtttttgattttaggacattctttcccttttttccctttatcagtgtcagcagtgttttacaaattttgttaatccttttgaaaactgggttttggttttgttaatcttctctattgtatacttgatttgtccattaatatttctgtccattatttcttgcttttatttttattgttgatttctttctacttactttgagtttaattggtattttttctgactttttgaagtgaaagtctatataattaattttcagcctttctccatttctaatacatatgtttaaacttatatgatttttgtaacattttatcttcattgtataagttttaacaagtatcttttgtcatttaattaaatttcattatgatttcttatgtgaataatggattatttcaaattatattttttattttccaatgtatgaggggatctactagttatcttcttgttaaaaaaattctggcatatactgtctgttcaatattatagtactttgaaaatttttgagacttgcttgctttttaaggtttgtagaatatctcttctatattctttttcttttattcttgttttctggttcatatatcttaactaattttactgtatcctttaatcccttttgcccttttctctttttattctttttttgtctcaatacttcagttggtaaattttcttctaattctttatgcctaccttgcagttaaatgtattcatttaattattaatttcagatatatatttttacatagcaaatctctttttgacttcttattgtattcattttactgtaaatcattcaatcttaccttttagctgtttgaacatattaaacatagtaatttaaaaatctctatgggtaactccagtataagtatgtgtttgtttctagtgtgtgctttttcctcttggttttctatcatgttgtttcatttacctccaaacatgaatgtgtttatgatgaatgagagtcactgaatatttaaaaaatcatagagatattttgaagctggaagaatgttcttttcatccagacaagatttattttgtttctgctatgcagctatggacactagcaattctcatttaccttaattcaatcaaggactgagaatactgaagtatgaaattaactctgtctgcttccagttcatacttcttccctgtacctcttttcttaaattttttttaaaattttatttcaacagcatttggagtataagtggtttttttttacgtggatgaattatatagtggtgaattctgagattttagtgcatccatcactcaagtagtgtacattgtatctaatatgtagttttttttaatccctagctcctcttccatcctctcctttctgagtctctaaagtccatcatatcagtctgtatgcctttgtgtactcatagcttagctcccacttataagtgagagcatatggtttttggttttctctgtagctctttagaatcccaaactgtagcctaagggaaaggtttccaaggtgctctccttattgcactccaaagtatgatttttatctccctaactctatgaatctagcaaacactttgcttaacttttcagcatctcaagtgccttttctgaatttgacagatacacgtcagaaatgtgctcccaaatgcctagcttatctctctttattaacttctccaaatctttgccaatagctatatgtcttaactgccttgtttgctctttagagctttgtaacacatgcatttttatagtttattctgcttttcaagtttttttcattgaaataattcttgtaatgaccaatagtctagtatgctgctgtaagacttctatagctgttaactcctttcatatttcaatttctttatgtgctgttttttgcaagaattcctaggctccattttctaattcatacgttggcaaatgatgaatgtgatatgacaatgatgacctctgttccagccatatacttttttaaagaaaattttattggaacacagtcatgctctcttgtttacatattatctatgacttcttttgtattacagtggcaaagttgagtaattgtggaagagaccatatggcctacaaaggctaaaatatttactatcttgttcattaagaaaaaatttgctgactcttattgagatttatttttcctttattcaactttctgaagtttgtcaattgatttaaaaattttaatgacttttcctttctaaattatatatttttatatctaacattattgtgccatttctatatttttgctatattttttgccttaaccaaacaatgtgttttaattgagtcagtgaataaagaactcactgaaagtagaagtggaaacctaagctataagctactatattatataagcttctcaacctataattgtttttccattaggtttgtaaaattagataatcctacatctcacattatgattctaatccttgtgttcggtaggtaataattgatctacaagagcaaggaaagtgaaaggaacagttagattcatgccatactctttgataaattctgaaatgaaacgtggggaacataaggattatgaggtttttatccagaacgtataggctgctttgagcaaagcaagttgagaaatatatgtgcagagatagagatgacaaaggagatggggatgtggagagagagagatcttatcatcagagctgctctgttttgacatatgacccaaagatcagacccttatatgacccttagaacttctaggtgtaattatgtgagagcttccagagcaagttaatgtgcagagaggataatttttcctcctcttcctctcatgttgccaactctgactcctaactgagcagctcagccctgggttatgcaagaaaactccatgtcttatttcaaaagtagacttggccacatttaaccaaacaagttttaaaaatgtattatgctatgtttatttcctataggtaagttggattcttgggctatctattaatcattttatttagaccaattgtataaagaatgctgacaaatatgtggtaaagataaaaatcatgccactggaatgattaaaaaagagttataatgttattgacataaaataacaaaagcactactaactatgaaactttaaatatccacctgatgacattgaccaatttgacttcatttccactttagaccaaaattttccaggtagggtctggataaccattttaggtaatttctctgaatcctttccttgagaaacagcttttgagaatcctcagtaaatgtcaaaaacaaactttctttttaaatttatagatagctacattgcatatattttattttgatttctccttaatgtacttttagtgaaaataataatttatgttcaatgtcactgatatttcttattacattcatgtgatctaagactaatagttgaaaaatggtttggttgcaggttaatatttaactttagtcagatataaaataatgcattttctttaagcacaaaatgtataactttagatatttcaaatcatattatagaagatctcattatcaaaataataattaagtattgaaaaaatacccttctcagggaagagaaagaagctctaggtgacttgagatgttctttatggtattctttattggctgttctgatgctgtatttaaccactatattttaacaggtaagttatttccctgaggattttattttatagattacaattattatattgcttatgtctttgcctttttctcttagggcaatcctaatatacaattaaatgctaaatcaaatggaaaataggagtaaaattttgatcagaaccacctccattgtgctatattatacagagaagctttcaaattttatggatggaagaagcagttatataaagaatactttttagtatttgtataaaaaacaacaaaaaattaaaaaccctatgaaaatctttgaccattatatatgatgttcattttactcatgtactacatgattttacctggtttaaaatgtttttctttttttgtaataaaataatgagaattatgtaaggtaattttttttaattacgagaccattctctaagacatggtcatgaaaagcaaaatagcaattcactttggtgggtcaactttgaaggagaacttgaagtgtaaatcttacaaaaactatcttatttacaaaaagatatacataaggaaataaatagtaatatagatttcttaattgttgctctaaagaactacaaattatgatgcagcacttgtctagaaaattctttcttgtttatgcttttcaatgttatcatgcacatgcaatcaaacaaaaaataataaagggaaagaatagaaaattttagaatcaggcttttttaatgattaccacaaattaatattgtcacttgttagggaatatgctgtgtattatcaatgcaaaatttagcataagacagcataataagacagtaatggttcattttagcttttgtgtcacattcaataactggaagaattttctaggactttcaagaatcacatcttatttgttgatgttggccagatactgtgctcttgagtggctttattttaatatattagtgtagtctcagaagccgtggcaaggtacggcagcacaaattaaattaattaggcattgattgaaatgtttctgtttgctaaatatttattcagacatagagacctaaatacaaataatgcttggtcccattacccagatatctcagagaccaatgcagataataaatctgtatcattcattgtgatatatgctataatagagatactactcaggacaaaatttctctttcttccttttaagttttaaattccaaaggtcttattttaagagaagatgtagatactgaactccaatgaaatgcaaatgttatttaaattgaagaaatatagggcagacttttatgagggaaattgaatattttattgcttaaaagactctttcctttgaataattgaagttgtaaagaaagcaaattaatgggtaaggaaactaggaagatgcatattggtgttcctgaaattttacaatgtactttaactctagtgcttagtataatttctttcatgttgaggcactggtaagtcctattctcctagataaaaatcttcagtgggattacgcctctgcgtttcatggcccaatgagagcttttgattttattacagattacaataagtcatagactgttctctcccttctggtttgagtgatactacacccttgccagcaccacagatggaaaaattgtaattaaagtgtctctgagaaatccttttctttgcaatcttcccaaatcgtccatatttttttgtgtatgttgaatgtatatctgaccatcaaataaaatactttcagaattgttctagaaaatatccttgcaataagattgaatgtgtttatctaggaaagaaagttctgttgtgcttctcaaagtgaaatttgtggaccccttgggttcccggagacattttaagggtatctctgtgttcaaaactatttttagaattattctaagttttttttgtcttttctagtgtattgacacttgaattaattacacaacatagttttacctgttggcacattagtatgaatcaaacggtggcaccaaacactactagtagtcactgtatttctcccaattactgcacttacaggaaaaaaaatgccagttttactccttgatgaatagtaacagttattggttttatttaaactccactttggaatacacatcattttgatattcagtgtgataaaatgggaagtgctcataaagtacttctaatgcatattgaaaattggcagttgtctttagaaaaagcactggagcagctgagttgttaactgaactttttttaaatgtgacatcatttttactggacagcacagacttactcattcatacttggatatttggcaggtatcttaatgcaaatgctcaagtgaccctactaataaagaacaaaaacaaaaactgacagtgtttgttgccaataacaaaatttgagcttttgagaaaaatcaaactttgagaaacctgtattcactattctgagcctgacagcttttcaacacttaaagacttatccaatgaaattaatggtggtattaacaaatgtgatgttttaatattgcatgatgaaatgtgtcaacattaggaagatctggataacccagtggacgaatgttttaagatgatcaataaattaggttaaaaaatcatgcatgagtaaaggatatattcaaagtataagacaaaccaatggatttaatgtggcagcatataaaaatgtcgcagattccacattgcaactaacctttaagaagttattacttgttgagctttgctatattacattgaggaatattcacaattacctgaaagctatacagtgaaatattacctccttttcatattatacatacatgtgagaggccatattttcttcacatacttcaattgaaacaacatatcaagagattgaattggagccacatatgagattacagttatattctttaatccagacattaaagagaattttactaataaaccaatgatttctgttttctgtaaatttttaaaaaaatgctttttaagtaaaaaatgttatttgatgaacatgtgacaggtttataattgaatttttaatgattaaaacaacacttaagagcaggaggggcagagcaagatggtcacataggtctctccagcaatcattcctccactgaaacatcaatttgaataattattagcacacaaaatatcacctcagtaaaccaggtgaaagattactgtacctagttctagcacaataataacaaaagatacattgaagagggtaggaaagatagttttacgttatctgcatcacccccctcaaccccagggagcatagtgtggagagaactgtcatctgctttggggaaaagagggaagtgagcacaggactttgcctggactccaatatcaggcctactgcagtaaaatccagcactggatagaacctcatggccccagactttaggctgttatttgacggctgagcctctagccccatgctggtgccaagtgagaccatgtggccctaggcttcaagcttgcatggtggactcagtccctggaccacaccatggatgggttattagtggcccaacctctgaacagcacttagtgacacggatgccgcagtggccctgagctttacgcatgcctcagtgctgcaccagtcacagtggtcccaggctttgggactatgcaaggcagcctgcccagaatttttggataggctgattgttgaaggacttttccagacaaaggcaatctgcaaagattggaataagtacctacttccagagatgtttatacattgacacattgtcacaagagtcaaaagcaatcagggtaacatgacgtcagtaaagagagaaaataacgtgccagtggccaatcctaaagaaatggagatgtatgaaccacccgaagaattcaaaataattattttaaggaagcacagcaaacttcaagaaaatacagagaaacaatttaacaaaatgagaaaaatgatgagtgatcagaataagaaatttaatagaaaggttgtaataattataaaaaagaaacaaatttcagagatgaaaaatacaatgggtgaaatgagaaatgaaatagagagcatcaacagcagaattgatcaagtagaagagtctgtgaacttaaaggtaggttatttgaaaatatagatagagaataaaaaaacagaatgaagaggaaggaagaaagcttatgggatttatgggacatcatcaaaaggacaaatattcaagttacaagggggaaaggagacaagaaattaaaagtaatagaaatcttaagtaaataaatagtagcaaaaaacttttaaaacctggaggatgatgtaaatatccaggtaaaactgagagaaaagtccccagtcagatttaatccaaagaagattaacccaagatatattaaaatcaaactgtaaaatatcaaagacaaagagaggattctgaaaactggaagataaaaaagcaaataacatattagaaagttttaatatgactagcagcagacttagcagaaactctgcaggccaagagagtaggatgaaatattcaaagtgctaaaagaaaaaacaaagaaacaaacaaacccatccaattgagaatattatacccagtaaagctgtgcttcagaaataaaggagggataaagattttcctggatgaacaaaagctgagggagttcattacaattatacctgtcttacaagaatgttaaagcgagtttttcaagctgaaagaaaaggatgctaataagtaatataaaaatatctgaaagtataaaactcactggtaaaactacagtaaaattcagaatactcatactataatgatggtgatgtttaaaagacaaaactgctaaaataataatagctataagattttgttaaaggacatgcaatatggaaagatgtaaattgtggtatcaaaggtgcaaactgtggggaggagtggagtaaaaatgtggagtgttttttttttctctgtaagtggagctgttattaacttaaaataaccagttacaaatatgtttattttttgtaagcatcatggttaagcacaaaacaaatactgatagtagatacacaaaatataaaaagcatggagtcaaaacataccattatatatatatatatgtgtgtgtgtgtgtgtgtgtatgtgtatatatatatatatatacacacacgttttacatgataaattacatagaaatttcttttttaattaaaaaggaatatttacatttttttcagttgtaatttccactattttaaatatccatagatataacccacataaacaacagatctttgggattctcaataacttttaagagtctaaaggggtcctgagaccaaactgtttgaggaccatggtgttcaaatattaaccaatctcttttcttcttattgtcatgtcttgaatgctgggtgatgaatgaacctttacacttaatgtatttttttaacaggtaagatttcttcaatatccaaaacatttcaaatcattttcttcagtatttttcattgaatttttaaccacataaggcaatttcaactcccataatgtggtttcaacatcaatcaacactattctactttgaatgaataagaattcatatgaaaaagtagagtgactattgttcttttctgtaacattgagaaataaagccaaaaggcaggattctactcatttgcattctagtaaaagatcaaggagatagtgtgtttttatcactctttacaataatgtaaactaatgatagtcacttaatcccttgcactttttgggttacatagacaaaatattggaacaagtaactattttgtgttgaaatgtcattttatactgtaaatgcttagatttcaccactaaatacctagattcaaaatttggctttgctactaacagatgtttacccgtaagttgcacacttctctctctcggtcttttttttttttttttcaggtgtgaaatattgctattaatagtgtctatctcatagggtggctaagatgattaaatgagatgatatagtttaagttctcaaaaaagccaacaatgattgttacctttcttttaggtgttgggtatcagcctcaatttctaaagaagaatctcttttgcctcccaattgtgctgaattggaaaccttacctatgtatttatttattcattcaaaaaccatctattataaaccatatttgtgccaaactctaagccagttactgaaaacacataagtcaataacagcacaatccttatcctccaggagttcataatccagtcagggaaaaggagacacacagataaagagaggagggatagagcgaagacattggagaaatcaggagcataccaacaccctaatttttcacagcagggagccagtcaattcagtccaacactgaaatacatagcttaataactacatgtttccaaaccattgtttcataatctatttccttaatcttagaaagattactgtcttgtggtaagaagacattaacttcaaatttggtatttcttttatttcactttagtttatttttcttctataaaatcaaaataaattacagtcttttaatttaaatagcattttcaacatatttttctttcttttattctctctatccagttcatttaagcatgcaaaatgcttagggaggagtcttaaattgtatttaacaaacgttaatggtgtttatttctggatactaggatttgaaattagcttttcaaaaatattatttaaactttcctgcaatacttacaatggataattatcatttttaccaaagcaataaagtgttttttttcctataagagagatataatggcattatgctcacagtggaaaggaagtaaagaggaggtgctactgtttggggaaagagtagctgaggagaaagagggagatcagtagttacagtattagaagcattaattgtgtctttaagggttaaacagaggctctctgatttctgaatgttaccttatgtttttataacaggtgagtctcactgaacttataaaaaaatttactttgaaataattatagatttgtaggaagttgcaaagagagtacagagatttcccatgtacctttcatcctatttccctggagtggtggccatcggagggagagatcattcacaggcatgactgaagaaagaccccaaatcctaatgttcagtctttaaagaatagactggccaaccatttttttttcgtgtgtgattttcctgaggctttagatagggctaaaacctatgtgggtagacagggaagatcgaaaccagaaaattgattattgttaacaatgtgtgtttatagttctatgtcattttatcacatgtgtaagtttatgtacccatcactgcaaccaaatattacatcactttgtagatttccctcatggcacccactattcctccaccatccttaactcttggcaaccactaatattttcttcatttccataattttgtcatttcgtgaatgttatacaaatggaatcatacagtatgtcaccttttgagactggcttttttgactcaacctaatatcctttgacatccatccaagatgtatgtatgtatttattgttcatttaaaaaattgtatagtattccatggtatagatataccacagtttaaccatgctctatcaaaaaatattccagtttttagctattgcaaacaaaactcctatcaagttttgtgtggatataagtttttattcctctggggtacatctccagaaatgtaatgctggatcataaagtaactgtatgtttagctttgaaagagatcaccaaactatactccagagggactgtaccattttacaatcccaccagcaatacatgagagatctattttttctgcattcttgctagtatttggtatcgttgctattaaaaattccttaactcttctaatagatgtatgctgatatttcatcagggtcttaatttgcattgcttaatgactaatgacattgaacatcttctcatgtgcttatttgccttctgtatagcttgtttagtgaaatgcctcttcacgtcttttgattattttctgattggatgatttgtgttttttagaagttgaatgttaaaagatctataaatcctaaatatgagtcaattgtcagatacattgtttgcggatagtttctcccagtctgtagttgtcttactattatgatgatttccatccctgccatctctcatctctccttttggaactctgggacatgaattctagatattttgttatagtctcacaatttatttatttattttttatatctatttgctctttatttttcagagtgggtaatttctattgttatatctttgaattcacttgttcatcactttgccctctccattctgcttttgagcatagctattgtttttcctatcttgggtattatggttttttagctctaaaatttcaagttgattctttttcaggtcttctatttctttgctgagacatcccacttccttcatttgtttcaagaatgttcctacttggttcttaagcatttttatgatggttgctttagaatccttgccaaataattctaacatctttgtcatctaattagggtcatgatcttctgattagcttttctcattcaagttgagaatttcctgggttttgatgtgacaaatgatttttaattgcatcttcgatattttaggtactttattttatgactctggatcttacatcttgtgttttagcaaacatattctgatactggtaagatggaaagtacaggtttcccataaggccttgtttgacacccttggagaaagggcactttcttactgtgccccatataggataccctgacatcacaggggctagaagcctccttgcatcgaaggttaatgaaggctaaagttccagcttctcacttgttctcctctgacacttccagagagggaaaagagcacctcattgctgctgattcggtggaagtctaggatccccaagtagcctcccttgacaccatcaagagggaccttgttagtatagtgcaggtataaatgtcctggctccctacatttttttcttctcttatactaccttggctaagggtgaaagttgggaaagggaaggacatatccatggatagggctaaggtgaattctgtggtgtttgactggggtagtgtggctattttctgaaagttttctgtcttgctacactgtcctttttctcatgctttgactagatgaaactagtcaacagcaaaaaaaattttcctttttgctggctctaatttgtattttccagttgtgagtgtctccaaaagccaatctgggacatatgaagtaaaaagaaaacctagagagctcatctctgtattgtttcttgggtctcaaggtctctagccaaattgcattatctgcacttttcaatctttatgtttgatttatgcataatgtccagagattttagctacatttagtgtaaagaagagggaaaagtgtgtctactccatttggtccagaactggaagtactctcactgaacttccaaaagattttaatataaagaattgttggggcatttatactccaaagcctcgttgcttactttatcagtagaaagatcacatatttaggttccgaaaagtgctatgccgtttaatgtatagagcatggtcttgcttaagtgaacctagtttttaaatagtagtaaactttgacctcgagaaaggtaatttaattgctctgaactttatctcctgttcttctaaaatggggataataagttttgcatctgaacttaataaactgtctaacaaaagtctgagtagtgaacattagatatacacaatgtaaatatataagcttatataagtacttaacagctctaaaattatggagggtttggggtaagacagaaatgctaagttttaaaatgacttttcaaggatgtatggcaacacattgtccttggcgtgctggatggcaatgcttaatgcaacttagtgtgctgacttaggacctctaaaaggacattgtattaattttgaaacagaagaattacattgcaacagaggttgaaaaaaattataggtgtcaactgagaactgctctctaccagaacctaggtattaattggccaactttgctagttattcctctgaaacctgaatgaagagaaggtagtaaaggaaatcatttagtaatggaaaaaataaacacaagattttagtaggaagaaggtactaaaagccctgttaaaagagtcctgggagcttccttgactggcatttgaaattaatcttatattttcctcataagcagttgttagcatagcagaattttgatttgtttagaagtcaaatgtgatttactaattcaatccctgtggtttgagggagaaaggagtaggtccctattagaactgtgaaatcagtacagtttgctctcataaatgctcatacacaaccctcctcacttcctctttttcttgtggttctttttagtccccaaagtccagcaaccccttttttccccttgaccaatttaaaacaaaccatttgaatggaatcgtagatgattgcaatttagtgtggatttagttgcattgaaaaatgctgtcacatgttggaaaaaaaagatcaaagatcatttctcctctagaaaagcttcaggctccatattgagatgtattggggatatttcattcttcagctctcaaaatcaccctatagagttgccttcacacatatttaataacttgttgacacattgctatttatgatataaaataactgatttatctatttgatataggtaaaaaatgctgatcataaccagatattattgtaatagtatcacaatcatacgtgtgtgtgtttgtgtgtgtctgtacgtgtatatgtgcttacagagtgtatttgcagggaaatgaagaatgggatcaattgcttgattaattcaaatttatatcacactttaaaactgcaatgatctgaattattgtatgttccgaagataacttattaagccattgcttttttggtttctttcttaaattgtatttaaaattggtcaaatttcaaatattaaatacaggacttacactttttaaatatactttccacaggtaatctggcccttttctccccctgtcatagatcactggtgccttttgaaaaatcctaagttatacatcagttattagatgactggggcccacctgcatgccctagtcctgaaagctacattaggatatatgtttcatttccactcttgtttgtttcattttcaggataagttgccttgattctgacatttggcccagcctgtactggtgtgccgcaatgagagtcaatctctattgacagcctgcttcagattttgcttttgttcgttttgccttctgtccttggaacagtcatatctcaagttcaaaggccaaaacctgagaagcggtgggctaagataggtcctactgcaaaccacccctccatatttccgtaccatttacaattcagtttctgtgacatctttttaaaccactggaggaaaaatgagatattctctaatttattcttctataacactctatatagagctatgtgagtactaatcacattgaataatagttataaaattattgtatagacatctgcttcttaaacagattgtgagttctttgagaaacagcgtggattttacttatctgtgtattcacagagcttagcacagtgcctggtaatgagcaagcatacttgccattacttttccttcccactctctccaacatcacattcactttaaatttttctgtatatagaaaggaaaactagcctgggcaacatgatgaaaccccatctccactgcaaaaaaaaaaaaaaaaaataagaaagaacaaaacaaaccccacaaaaattagctgggtatgatggcacgtgcctgtagtcccagttactcaggatgattgattgagccttggaggtggaggctacagtgagctgagattgtgccactgtactctagccagggagaaagagtgagatcctggctcaaaaaaaccaaataaaacaaaacaaacaaacgaaaaacagaaaggaagactgaaagagaatgaaaagctggggagaggaaataaaaataaagaaggaagagtgtttcatttatatctgaatgaaaatatgaatgactctaagtaattgaattaattaaaatgagccaacttttttttaacaatttacattttatttctatgggaaaaaataaatattcctcttctaacaaacccatgcttgattttcattaattgaattccaaatcatcctagccatgtgtccttccatttaggttactggggcaaatcagtaagaaagttcttatatttatgctccaaataattctgaagtcctcttactagctgtgaaagctagtactattaagaaagaaaacaaaattcccaaaagatagctttcacttttttttttccttaaagacttcctaattctcttctccaaattcttagtcttcttcaaaataatatgctttggttcaatagttatccacattctgacagtctaatttagttttaatcagaattatactcatcttttgggtagtcatagatattaagaaagcaagagtttcttatgtccagttatggaatatttcctaaagcaaggctgcaggtgaagttgtgctcaagtgaatgttcaggagacacaattcagtggaagaaattaagtctttaaaaaagacctaggaataggagaaccatggaaattgaggaggtaggcctacaagtagatattgggaacaaaattagagaggcaaccagaaaaagttattttaggctcaccagagttgttcttattgcacagtaacacaccaatataccaaaacagcaggtattgcagtagagaaagagtttaataattgaatggcagaaaaatgaggaaggttgaggaaacctcaaatctacctccctgctgagtctaagtttaggatttttaagagaaaggcaggtaaggtgctgaaggtctggagctgctgatttgttggggtatagggaatgaaatgaaacatacagagatgaaaactggaagtttttttttgtttgttttgttttttttttgttgttgtttttttttttttttgtttttttgctgagtcaattccttggagggggtcttcagactgactggtgtcagcagacccatgggattccaagatctggaaaactttttagatagaaacttgatgtttcttaacgttacatatattatcttatagaaataactaagggaagttagtgccttgtgaccacatctatgtgacttttaggcagtaagaaactataaggaaaggagctaacagtcatgctgtaagtagctacagggaattggcttaaagggcaagttggttagtacttagctgtgtttttattcaaagtctacattttatgtagtggttaatgtttgctgttcattaggatggtttcacagttaccatacaaatgtagaagcaacaggtccaaaaagtagggcatgattttctccatgtaatccagggagaaaacaagccatgaccattgttggttgggagactgaaggtgattgaaggttcaccatcatcctcaccaacttttgggccataattcacccaaccctttggtggagcctgaaaaaaatctgggcagaatgtaggacttctttattttgtttaaaggggtaacacagagtgcccttatgaaggagttggagatcctgcaaggaagagaaggagtgaaggagagatcaagagagagaaacaatgaggaacatttcatttgacccaacatcctttaggagcataaatgttgacactaagttatcccttttgtgctaaaatggacagtattggcaaaatgataccacaacttcttattctctggctctatattgctttggaaacacttaaacatcaaatggagttaaatacatatttgaaatttaggttaggaaatattggtgaggaggcctcaaaaagggggaaacatcttttgtctgggaggatattttccattttgtggatttccctgatctttttctaccaccctgaggggtggtgggaattatcattttgctacattttagaggtcatccaggatttttgaaactttacattctttacggttaagcaagatgtacagctcagtcaaagacactaaattcttcttagaaaaatagtgctaaggagtatagcagatgacctatatgtgtgttggctgggagaatatcatcttaaagtgagagtgatgttgtggagacagttgaaatgtcaatgctagagcctctgtggtgtgaatgggcacgttaggttgttgcattagaaagtgactgtttctgacagaaatttgtagctttgtgcaaactcacccaccatctacctcaataaaatatagagaaaagaaaaatagagcagtttgagttctatgaggtatgcaggcccagagagacataagtatgttcctttagtcttgcttcctgtgtgccacactgcccctccacaaccatagctgggggcaattgtttaaagtcattttgttcccgactagctgccttgcacattatcttcattttcctggaatttgatacagagagcaatttatagccaattgatagcttatgctgtttcaatgtaaattcgtggtaaataacttaggaactgcctcttctttttctttgaaaacctacttataactgttgctaataagaatgtgtattgttcaggacaacttgtctccatacagttgggttgtaaccctcatgcttggcccaaataaactctctacttatatcagtttttcctacacttcttccttttaggtcaacaataccaagaggggttactgtgctgggtaatgtgtaaacttgtgtcttgtttagaaagataaatttaaagactatcacattgctttttcataaaacaagacaggtctacaattaatttattttgacgcaaattgataggggggccaagtaagccccatatgcttaatgatcagctgatgaataatcatctcctagcaacataactcaatctaatgctaaggtacccacaagatggcaaggctgatcaaagtcgtcatggaatcctgcaaccaaaagccatgggaatttggaagccctcaaatcccattcctaatctgatgagtctatggaccaatttgtggaggacagtagattaaatagatctgatttttgccatcaatgtaaggaggataaaaacttgcataccaattgtacacccttgcaaaatctttctctgatgttggagaaaatgggccagtgagatcatggatatagaagtacagtcaatgttcagctgtaccctcccacaatcccacttccttcctcaacacaattcaaacaaatagactcagactgtttcaggctccaggacaggaagtgcagtgtaggcaaaattgcaaaaattgagggcacaggggtggaggtgggggggttgaataacaagctgtgctaaataattacgtgtaaatatattttttcatttttaaaaattgatttcttttgcacattccatgacaatatatgtcacatttttaaaataaatgcaaagaagcatacatccaagctgccagctgagtttttttgctgctttgagtctcagttttctttctttcctagagtctctgaagccacagatctcttaagaactttctgtctccaaaccgtggctgctcgataaatcagacagaacagttaatcctcaatttaagcctgatctaacccctagaaacagatatagaacagctgccagctgagtttttttgctgctttgagtctcagttttctttctttcctagagtctctgaagccacagatctcttaagaactttctgtctccaaaccgtggctgctcgataaatcagacagaacagttaatcctcaatttaagcctgatctaacccctagaaacaggtaagcgactttttaattgaaacatagtatttgtacgtatttatggggttatgtgtgatattttgatacaagcatacaatgtaatgaccaaatcaggatcattgggaaatccatcacctcaaccatttatcatttctttgtatttggaacattccaaattttctcttctagctatttcaaaatagacaataaattattgttaactatagttaaactgttgtgctatgaacacaagaacttattccttctatgtagctgtatttttgtaaccattaaccaacctcttttcatcatctccttcctctgactttcccaacctctggtaaccaccatgctactctctgcctccatgaaatcaacttttattttaagcttccacgtgtgagtgagaacatcacaggtaagtgacttcttgccatccaattttgctagctgtgtgtgaagaaaaaagcttgctttctttttttctaaaaaggagtttcagagtggaattgctgctaatactttgctctttcatttgtcttttattttaatgaaaatttcacacacagataactagagagtataaatgaaccatactgtaatctgatatagttttatccaattttaaaaatgatttgctttttaaattagaatagttttcttttacttaaatacaaaagcattacaaataaagttgaagaaatctatgactctctactatatattgttttcttatgagatggagtctcactctattgcccaggctggagagcagtgtctcgatgtcggctcactgcaacctcagcctcctgggttcaagggattcttgtgcctcagcctcccaagtacctgggattacaggcgtgcaccagcatgcctggctaatttttgtatttttagtagagacgaggtttcaccatgttggccaggctggtcttgaactcctgaccgcaagtgatctgccagcctcagcctcccaaagtgctgggattacaggtgtgagccaccacacctagcctctcctatattctttacctttctttttatttccagaaggcaacattatctagactttggtataaattattgtcataattgtttttatggttttctgtatgtgtgtatatatttatctaaatatgatctctagtataatttgttaaaattacttctgtttttatataccagcaaaaatggttttacacaataacttaaaaaattaatatacttatattaattttatttttattgatacataatacattacatatttatggggtacaggtgatatttggtgatgcacttagaatgtgtaatgatcaagtcagggtatttgtggtttccatcgctttgagtatttattatttccatgtgctgggaacaacccaagtcttctagctactttgaaatagacaatacattgcttttggccatagtcactctactttgttgttgactaatagaacttctaccttctatttaactgtatatttgtactcattaacctacatctcttcatctctccctcctagacacccacccacccttcctagcctccagtatttatcattatactatccacatttataagatcaacatttttagctgatctaaaatgatgagtgagaacgtgtgatatttcctgtgcctaggttatttcacttaatattctccagttccgtccatgttgctgcaaatgacatgattttactgtttttatagctaaatagtattccattgtgtaatataccacattttctttatccatccacttatggacagttaggttgattccatatcttttctattgttaatagaaattcacaatagaaaggttgctgtgataaacctgagagacaccagaaggaattttaacatattgaccatactaaacaatatttaacatattgattgtattcagctatcttttacaatgtggtgtacagactctaaaatagctcctaattgtccctgtcctattttttttttaatactcatgtccgtgtataatccccccttgtctgtggatggaaactgtgacttaacggtaacaaatagaatttggcaaatgtgatatgttaagattataatgtctgctatgctaggagattctctcccttgctggtttcaatgaagtaagtggtcatgttggggaggcccatttggcaaagaactaagggtgacttcaggccaatgactaactgagaactgaggataacctctgatcattagctagcaagaaatggagttctcatatctacaaccataaggaactgaattctgctaacaaccataggagcttggaagcatgtccttctcccgttaaacattcagaagagtctgcagctgtggctcgcactttgataactgcctcatgaaaaattctgaagcagagaaccaaactggatttctgacccagagaaactgtgagactataaatgtgtgttgttttaagtctctaaacgtatgagaaattgctatgcagcaatagataaatagcacactaaattagttaatactattactttatcggtagatgctttaaggttttccacatataagataatatcatctgtgagcagagatgattatacttcctttataattcaggtaccttttcctttttcactttcttttttattttggcctacttgttctggctaggacattcagtattatgttgaatagaagtggtaaaagtggataatcttgtcttgtactttatcttagaggaaaagctgtcagtttttcactgctgaatatgatgttaactatgaactttttatacatgtatttactatgttgaggtaatttccttctactcctggtttaagtgttttttgttttttttttttttttttttttttttttttaaatcatggaaggacttgggttttatcaaatgtcttttctgtatctattgagatgaccaatttgtattagtcagcgttcttcagagaaactgaaccaacataaaaaaaataaaattaaaaaaaaactaaggaaatttgttatgggaggtggctcatgtggtgttggagggcgagaagtctcactatctgccacctgccagatgtaaagccaggaaagctggtggtgtaattcagtctgaatccaaatgcctgagaactggtggagccagtggtggaactcccagtctgaaatcaaagtcctgggaactgtgggaactgagagagctggaggtgtaagtcccagaatccgaatgtttgagaaccaggagctcagatatctgagagcagaagaagatggatactccagctcaagaatagagaatttgctcttcctctgcctttttgctctatttgggccctcaatggattggatgatgtcagctcatgttggatcttttttatgcagtttactaattcaaatgctaatctaaaatgtgtttgtatattcatttgcctcaacatttcttttcttttctttttttcctttcttttctttttttgagatggagtgtctctctgtcacccaggctggagtgcagtggtgcaatctctgcctcccaggttcaagcgattctcctacttcagccttctgagtagctgggactacaggtgcacaccaccacacccaatttttgtatttttgtatttttgttagagacggggcttttccgtattggccaggctggtctcagactcatgacctcaagtgttccgccgaactcggcctcccaaagtactgggtttacaggtgtgagtcaccacgcctggcctcaagatatttttaaaattcccttttgatttcattttgatccactgcttattccagagggtgtagtttaattctcacatccttgttaattttctagattttctgatattgatttctagtttcattacatggttatgaggaaagacttgatatggtttcaatcttcttagatttgttaagacttgttttttgacctaacatgtaatctatcctggagaacgctcctataatacacttgagaagaatgtgtattttgttgttgctgggtggaatgccctgtatatgcctattaggtccattgggactatagtgttcaagttttctgttttcctattgatcttctgtttggatattttataatggataaagtattgaaagtgggctatcaaaatctccttctcttattgtgttgctgtttctcccttcaattctttcagtgtttgcttcatttatttaggtgctctgatgttggatgaacatatatttataacggttatatttttctggagaattgacccttttcttattatatgatgtccttcatagcctgttatgacaggttttgatttaatgtctattttgtgtgggataaggacacacaccccttgcgggttatcttgcggttcttgcagttaccatttgcaaaggtacccttattatcacttgattttcatcctatgtgtgttcttaagtctaagtgagttcttggggacagcatgctgttgtattttgtcatgacatgctttgactcagtattatccttctttctttccttccttttttttttttggtttgctaatattttgctgaggatcattccatctatatttataaaagagattggcctgtaatttttcttgcttataacgccattaacaggttttggtatctaagttattctctggaagaacatgtgtaagattgtgtattatttattcttcaaaatttggtagaattcagcagctagactctgatccttgagttttcttggggaagtcttaaattaattatgaatttagtttttaaaaatagctatgagatagtcaaattttgtatttacttttatgtcagctttggtaagttgtatttttctagaaatttgtccacttattctcaaatttaattttacaaagttgtttatcttcagaccattttatcgtttatcatttattgcatctggactgatgttttctcttacgtttttgattttaggacattctttcccttttttccctttatcagtgtcagcagtgttttacaaattttgttaatccttttgaaaactgggttttggttttgttaatcttctctattgtatacttgatttgtccattaatatttctgtccattatttcttgcttttatttttattgttgatttctttctacttactttgagtttaattggtattttttctgactttttgaagtgaaagtctatataattaattttcagcctttctccatttctaatacatatgtttaaacttatatgatttttgtaacattttatcttcattgtataagttttaacaagtatcttttgtcatttaattaaatttcattatgatttcttatgtgaataatggattatttcaaattatattttttattttccaatgtatgaggggatctactagttatcttcttgttaaaaaaattctggcatatactgtctgttcaatattatagtactttgaaaatttttgagacttgcttgctttttaaggtttgtagaatatctcttctatattctttttcttttattcttgttttctggttcatatatcttaactaattttactgtatcctttaatcccttttgcccttttctctttttattctttttttgtctcaatacttcagttggtaaattttcttctaattctttatgcctaccttgcagttaaatgtattcatttaattattaatttcagatatatatttttacatagcaaatctctttttgacttcttattgtattcattttactgtaaatcattcaatcttaccttttagctgtttgaacatattaaacatagtaatttaaaaatctctatgggtaactccagtataagtatgtgtttgtttctagtgtgtgctttttcctcttggttttctatcatgttgtttcatttacctccaaacatgaatgtgtttatgatgaatgagagtcactgaatatttaaaaaatcatagagatattttgaagctggaagaatgttcttttcatccagacaagatttattttgtttctgctatgcagctatggacactagcaattctcatttaccttaattcaatcaaggactgagaatactgaagtatgaaattaactctgtctgcttccagttcatacttcttccctgtacctcttttcttaaattttttttaaaattttatttcaacagcatttggagtataagtggtttttttttacgtggatgaattatatagtggtgaattctgagattttagtgcatccatcactcaagtagtgtacattgtatctaatatgtagttttttttaatccctagctcctcttccatcctctcctttctgagtctctaaagtccatcatatcagtctgtatgcctttgtgtactcatagcttagctcccacttataagtgagagcatatggtttttggttttctctgtagctctttagaatcccaaactgtagcctaagggaaaggtttccaaggtgctctccttattgcactccaaagtatgatttttatctccctaactctatgaatctagcaaacactttgcttaacttttcagcatctcaagtgccttttctgaatttgacagatacacgtcagaaatgtgctcccaaatgcctagcttatctctctttattaacttctccaaatctttgccaatagctatatgtcttaactgccttgtttgctctttagagctttgtaacacatgcatttttatagtttattctgcttttcaagtttttttcattgaaataattcttgtaatgaccaatagtctagtatgctgctgtaagacttctatagctgttaactcctttcatatttcaatttctttatgtgctgttttttgcaagaattcctaggctccattttctaattcatacgttggcaaatgatgaatgtgatatgacaatgatgacctctgttccagccatatacttttttaaagaaaattttattggaacacagtcatgctctcttgtttacatattatctatgacttcttttgtattacagtggcaaagttgagtaattgtggaagagaccatatggcctacaaaggctaaaatatttactatcttgttcattaagaaaaaatttgctgactcttattgagatttatttttcctttattcaactttctgaagtttgtcaattgatttaaaaattttaatgacttttcctttctaaattatatatttttatatctaacattattgtgccatttctatatttttgctatattttttgccttaaccaaacaatgtgttttaattgagtcagtgaataaagaactcactgaaagtagaagtggaaacctaagctataagctactatattatataagcttctcaacctataattgtttttccattagatatagaacaatggaagtgacaacaagattgacatggaatgatgaaaatcatctgcgcaagctgcttggaaatgtttctttgagtcttctctataagtctagtgttcatggaggtagcattgaagatatggttgaaagatgcagccgtcagggatgtactataacaatggcttacattgattacaatatgattgtagcctttatgcttggaaattatattaatttacatgaaagttctacagagccaaatgattccctatggttttcacttcaaaagaaaaatgacaccactgaaatagaaactttactcttaaatacagcaccaaaaattattgatgagcaactggtgtgtcgtttatcgaaaacggatattttcattatatgtcgagataataaaatttatctagataaaatgataacaagaaacttgaaactaaggttttatggccaccgtcagtatttggaatgtgaagtttttcgagttgaaggtttgtaaaattagataatcctacatctcacattatgattctaatccttgtgttcggtaggtaataattgatctacaagagcaaggaaagtgaaaggaacagttagattcatgccatactctttgataaattctgaaatgaaacgtggggaacataaggattatgaggtttttatccagaacgtataggctgctttgagcaaagcaagttgagaaatatatgtgcagagatagagatgacaaaggagatggggatgtggagagagagagatcttatcatcagagctgctctgttttgacatatgacccaaagatcagacccttatatgacccttagaacttctaggtgtaattatgtgagagcttccagagcaagttaatgtgcagagaggataatttttcctcctcttcctctcatgttgccaactctgactcctaactgagcagctcagccctgggttatgcaagaaaactccatgtcttatttcaaaagtagacttggccacatttaaccaaacaagttttaaaaatgtattatgctatgtttatttcctataggaattaaggataacctagacgacataaagaggataattaaagccagagagtaagttggattcttgggctatctattaatcattttatttagaccaattgtataaagaatgctgacaaatatgtggtaaagataaaaatcatgccactggaatgattaaaaaagagttataatgttattgacataaaataacaaaagcactactaactatgaaactttaaatatccacctgatgacattgaccaatttgacttcatttccactttagaccaaaattttccaggtagggtctggataaccattttaggtaatttctctgaatcctttccttgagaaacagcttttgagaatcctcagtaaatgtcaaaaacaaactttctttttaaatttatagatagctacattgcatatattttattttgatttctccttaatgtacttttagtgaaaataataatttatgttcaatgtcactgatatttcttattacattcatgtgatctaagactaatagttgaaaaatggtttggttgcaggttaatatttaactttagtcagatataaaataatgcattttctttaagcacaaaatgtataactttagatatttcaaatcatattatagaagatctcattatcaaaataataattaagtattgaaaaaatacccttctcagggaagagaaagaagctctaggtgacttgagatgttctttatggtattctttattggctgttctgatgctgtatttaaccactatattttaacaggcacagaaataggcttctagcagacatcagagactataggccctatgcagacttggtttcagaaattcgtattcttttggtgggtccagttgggtctggaaagtccagttttttcaattcagtcaagtctatttttcatggccatgtgactggccaagccgtagtggggtctgatatcaccagcataaccgagcgggtaagttatttccctgaggattttattttatagattacaattattatattgcttatgtctttgcctttttctcttagggcaatcctaatatacaattaaatgctaaatcaaatggaaaataggagtaaaattttgatcagaaccacctccattgtgctatattatacagagaagctttcaaattttatggatggaagaagcagttatataaagaatactttttagtatttgtataaaaaacaacaaaaaattaaaaaccctatgaaaatctttgaccattatatatgatgttcattttactcatgtactacatgattttacctggtttaaaatgtttttctttttttgtaataaaataatgagaattatgtaaggtaattttttttaattacgagaccattctctaagacatggtcatgaaaagcaaaatagcaattcactttggtgggtcaactttgaaggagaacttgaagtgtaaatcttacaaaaactatcttatttacaaaaagatatacataaggaaataaatagtaatatagatttcttaattgttgctctaaagaactacaaattatgatgcagcacttgtctagaaaattctttcttgtttatgcttttcaatgttatcatgcacatgcaatcaaacaaaaaataataaagggaaagaatagaaaattttagaatcaggcttttttaatgattaccacaaattaatattgtcacttgttagggaatatgctgtgtattatcaatgcaaaatttagcataagacagcataataagacagtaatggttcattttagcttttgtgtcacattcaataactggaagaattttctaggactttcaagaatcacatcttatttgttgatgttggccagatactgtgctcttgagtggctttattttaatatattagtgtagtctcagaagccgtggcaaggtacggcagcacaaattaaattaattaggcattgattgaaatgtttctgtttgctaaatatttattcagacatagagacctaaatacaaataatgcttggtcccattacccagatatctcagagaccaatgcagataataaatctgtatcattcattgtgatatatgctataatagagatactactcaggacaaaatttctctttcttccttttaagttttaaattccaaaggtcttattttaagagaagatgtagatactgaactccaatgaaatgcaaatgttatttaaattgaagaaatatagggcagacttttatgagggaaattgaatattttattgcttaaaagactctttcctttgaataattgaagttgtaaagaaagcaaattaatgggtaaggaaactaggaagatgcatattggtgttcctgaaattttacaatgtactttaactctagtgcttagtataatttctttcatgttgaggcactggtaagtcctattctcctagataaaaatcttcagtgggattacgcctctgcgtttcatggcccaatgagagcttttgattttattacagattacaataagtcatagactgttctctcccttctggtttgagtgatactacacccttgccagcaccacagatggaaaaattgtaattaaagtgtctctgagaaatccttttctttgcaatcttcccaaatcgtccatatttttttgtgtatgttgaatgtatatctgaccatcaaataaaatactttcagaattgttctagaaaatatccttgcaataagattgaatgtgtttatctaggaaagaaagttctgttgtgcttctcaaagtgaaatttgtggaccccttgggttcccggagacattttaagggtatctctgtgttcaaaactatttttagaattattctaagttttttttgtcttttctagtgtattgacacttgaattaattacacaacatagttttacctgttggcacattagtatgaatcaaacggtggcaccaaacactactagtagtcactgtatttctcccaattactgcacttacaggaaaaaaaatgccagttttactccttgatgaatagtaacagttattggttttatttaaactccactttggaatacacatcattttgatattcagtgtgataaaatgggaagtgctcataaagtacttctaatgcatattgaaaattggcagttgtctttagaaaaagcactggagcagctgagttgttaactgaactttttttaaatgtgacatcatttttactggacagcacagacttactcattcatacttggatatttggcaggtatcttaatgcaaatgctcaagtgaccctactaataaagaacaaaaacaaaaactgacagtgtttgttgccaataacaaaatttgagcttttgagaaaaatcaaactttgagaaacctgtattcactattctgagcctgacagcttttcaacacttaaagacttatccaatgaaattaatggtggtattaacaaatgtgatgttttaatattgcatgatgaaatgtgtcaacattaggaagatctggataacccagtggacgaatgttttaagatgatcaataaattaggttaaaaaatcatgcatgagtaaaggatatattcaaagtataagacaaaccaatggatttaatgtggcagcatataaaaatgtcgcagattccacattgcaactaacctttaagaagttattacttgttgagctttgctatattacattgaggaatattcacaattacctgaaagctatacagtgaaatattacctccttttcatattatacatacatgtgagaggccatattttcttcacatacttcaattgaaacaacatatcaagagattgaattggagccacatatgagattacagttatattctttaatccagacattaaagagaattttactaataaaccaatgatttctgttttctgtaaatttttaaaaaaatgctttttaagtaaaaaatgttatttgatgaacatgtgacaggtttataattgaatttttaatgattaaaacaacacttaagagcaggaggggcagagcaagatggtcacataggtctctccagcaatcattcctccactgaaacatcaatttgaataattattagcacacaaaatatcacctcagtaaaccaggtgaaagattactgtacctagttctagcacaataataacaaaagatacattgaagagggtaggaaagatagttttacgttatctgcatcacccccctcaaccccagggagcatagtgtggagagaactgtcatctgctttggggaaaagagggaagtgagcacaggactttgcctggactccaatatcaggcctactgcagtaaaatccagcactggatagaacctcatggccccagactttaggctgttatttgacggctgagcctctagccccatgctggtgccaagtgagaccatgtggccctaggcttcaagcttgcatggtggactcagtccctggaccacaccatggatgggttattagtggcccaacctctgaacagcacttagtgacacggatgccgcagtggccctgagctttacgcatgcctcagtgctgcaccagtcacagtggtcccaggctttgggactatgcaaggcagcctgcccagaatttttggataggctgattgttgaaggacttttccagacaaaggcaatctgcaaagattggaataagtacctacttccagagatgtttatacattgacacattgtcacaagagtcaaaagcaatcagggtaacatgacgtcagtaaagagagaaaataacgtgccagtggccaatcctaaagaaatggagatgtatgaaccacccgaagaattcaaaataattattttaaggaagcacagcaaacttcaagaaaatacagagaaacaatttaacaaaatgagaaaaatgatgagtgatcagaataagaaatttaatagaaaggttgtaataattataaaaaagaaacaaatttcagagatgaaaaatacaatgggtgaaatgagaaatgaaatagagagcatcaacagcagaattgatcaagtagaagagtctgtgaacttaaaggtaggttatttgaaaatatagatagagaataaaaaaacagaatgaagaggaaggaagaaagcttatgggatttatgggacatcatcaaaaggacaaatattcaagttacaagggggaaaggagacaagaaattaaaagtaatagaaatcttaagtaaataaatagtagcaaaaaacttttaaaacctggaggatgatgtaaatatccaggtaaaactgagagaaaagtccccagtcagatttaatccaaagaagattaacccaagatatattaaaatcaaactgtaaaatatcaaagacaaagagaggattctgaaaactggaagataaaaaagcaaataacatattagaaagttttaatatgactagcagcagacttagcagaaactctgcaggccaagagagtaggatgaaatattcaaagtgctaaaagaaaaaacaaagaaacaaacaaacccatccaattgagaatattatacccagtaaagctgtgcttcagaaataaaggagggataaagattttcctggatgaacaaaagctgagggagttcattacaattatacctgtcttacaagaatgttaaagcgagtttttcaagctgaaagaaaaggatgctaataagtaatataaaaatatctgaaagtataaaactcactggtaaaactacagtaaaattcagaatactcatactataatgatggtgatgtttaaaagacaaaactgctaaaataataatagctataagattttgttaaaggacatgcaatatggaaagatgtaaattgtggtatcaaaggtgcaaactgtggggaggagtggagtaaaaatgtggagtgttttttttttctctgtaagtggagctgttattaacttaaaataaccagttacaaatatgtttattttttgtaagcatcatggttaagcacaaaacaaatactgatagtagatacacaaaatataaaaagcatggagtcaaaacataccattatatatatatatatgtgtgtgtgtgtgtgtgtgtatgtgtatatatatatatatatacacacacgttttacatgataaattacatagaaatttcttttttaattaaaaaggaatatttacatttttttcagttgtaatttccactattttaaatatccatagatataacccacataaacaacagatctttgggattctcaataacttttaagagtctaaaggggtcctgagaccaaactgtttgaggaccatggtgttcaaatattaaccaatctcttttcttcttattgtcatgtcttgaatgctgggtgatgaatgaacctttacacttaatgtatttttttaacagtataggatatattctgttaaagatggaaaaaatggaaaatctctgccatttatgttgtgtgacactatggggctagatggggcagaaggagcaggactgtgcatggatgacattccccacatcttaaaaggttgtatgccagacagatatcaggtaagatttcttcaatatccaaaacatttcaaatcattttcttcagtatttttcattgaatttttaaccacataaggcaatttcaactcccataatgtggtttcaacatcaatcaacactattctactttgaatgaataagaattcatatgaaaaagtagagtgactattgttcttttctgtaacattgagaaataaagccaaaaggcaggattctactcatttgcattctagtaaaagatcaaggagatagtgtgtttttatcactctttacaataatgtaaactaatgatagtcacttaatcccttgcactttttgggttacatagacaaaatattggaacaagtaactattttgtgttgaaatgtcattttatactgtaaatgcttagatttcaccactaaatacctagattcaaaatttggctttgctactaacagatgtttacccgtaagttgcacacttctctctctcggtcttttttttttttttttcaggtgtgaaatattgctattaatagtgtctatctcatagggtggctaagatgattaaatgagatgatatagtttaagttctcaaaaaagccaacaatgattgttacctttcttttaggtgttgggtatcagcctcaatttctaaagaagaatctcttttgcctcccaattgtgctgaattggaaaccttacctatgtatttatttattcattcaaaaaccatctattataaaccatatttgtgccaaactctaagccagttactgaaaacacataagtcaataacagcacaatccttatcctccaggagttcataatccagtcagggaaaaggagacacacagataaagagaggagggatagagcgaagacattggagaaatcaggagcataccaacaccctaatttttcacagcagggagccagtcaattcagtccaacactgaaatacatagcttaataactacatgtttccaaaccattgtttcataatctatttccttaatcttagaaagattactgtcttgtggtaagaagacattaacttcaaatttggtatttcttttatttcactttagtttatttttcttctataaaatcaaaataaattacagtcttttaatttaaatagcattttcaacatatttttctttcttttattctctctatccagttcatttaagcatgcaaaatgcttagggaggagtcttaaattgtatttaacaaacgttaatggtgtttatttctggatactaggatttgaaattagcttttcaaaaatattatttaaactttcctgcaatacttacaatggataattatcatttttaccaaagcaataaagtgttttttttcctataagagagatataatggcattatgctcacagtggaaaggaagtaaagaggaggtgctactgtttggggaaagagtagctgaggagaaagagggagatcagtagttacagtattagaagcattaattgtgtctttaagggttaaacagaggctctctgatttctgaatgttaccttatgtttttataacagtttaattcccgtaaaccaattacacctgagcattctacttttatcacctctccatctctgaaggacaggattcactgtgtggcttatgtcttagacatcaactctattgacaatctctactctaaaatgttggcaaaagtgaagcaagttcacaaagaagtattaaactgtggtgagtctcactgaacttataaaaaaatttactttgaaataattatagatttgtaggaagttgcaaagagagtacagagatttcccatgtacctttcatcctatttccctggagtggtggccatcggagggagagatcattcacaggcatgactgaagaaagaccccaaatcctaatgttcagtctttaaagaatagactggccaaccatttttttttcgtgtgtgattttcctgaggctttagatagggctaaaacctatgtgggtagacagggaagatcgaaaccagaaaattgattattgttaacaatgtgtgtttatagttctatgtcattttatcacatgtgtaagtttatgtacccatcactgcaaccaaatattacatcactttgtagatttccctcatggcacccactattcctccaccatccttaactcttggcaaccactaatattttcttcatttccataattttgtcatttcgtgaatgttatacaaatggaatcatacagtatgtcaccttttgagactggcttttttgactcaacctaatatcctttgacatccatccaagatgtatgtatgtatttattgttcatttaaaaaattgtatagtattccatggtatagatataccacagtttaaccatgctctatcaaaaaatattccagtttttagctattgcaaacaaaactcctatcaagttttgtgtggatataagtttttattcctctggggtacatctccagaaatgtaatgctggatcataaagtaactgtatgtttagctttgaaagagatcaccaaactatactccagagggactgtaccattttacaatcccaccagcaatacatgagagatctattttttctgcattcttgctagtatttggtatcgttgctattaaaaattccttaactcttctaatagatgtatgctgatatttcatcagggtcttaatttgcattgcttaatgactaatgacattgaacatcttctcatgtgcttatttgccttctgtatagcttgtttagtgaaatgcctcttcacgtcttttgattattttctgattggatgatttgtgttttttagaagttgaatgttaaaagatctataaatcctaaatatgagtcaattgtcagatacattgtttgcggatagtttctcccagtctgtagttgtcttactattatgatgatttccatccctgccatctctcatctctccttttggaactctgggacatgaattctagatattttgttatagtctcacaatttatttatttattttttatatctatttgctctttatttttcagagtgggtaatttctattgttatatctttgaattcacttgttcatcactttgccctctccattctgcttttgagcatagctattgtttttcctatcttgggtattatggttttttagctctaaaatttcaagttgattctttttcaggtcttctatttctttgctgagacatcccacttccttcatttgtttcaagaatgttcctacttggttcttaagcatttttatgatggttgctttagaatccttgccaaataattctaacatctttgtcatctaattagggtcatgatcttctgattagcttttctcattcaagttgagaatttcctgggttttgatgtgacaaatgatttttaattgcatcttcgatattttaggtactttattttatgactctggatcttacatcttgtgttttagcaaacatattctgatactggtaagatggaaagtacaggtttcccataaggccttgtttgacacccttggagaaagggcactttcttactgtgccccatataggataccctgacatcacaggggctagaagcctccttgcatcgaaggttaatgaaggctaaagttccagcttctcacttgttctcctctgacacttccagagagggaaaagagcacctcattgctgctgattcggtggaagtctaggatccccaagtagcctcccttgacaccatcaagagggaccttgttagtatagtgcaggtataaatgtcctggctccctacatttttttcttctcttatactaccttggctaagggtgaaagttgggaaagggaaggacatatccatggatagggctaaggtgaattctgtggtgtttgactggggtagtgtggctattttctgaaagttttctgtcttgctacactgtcctttttctcatgctttgactagatgaaactagtcaacagcaaaaaaaattttcctttttgctggctctaatttgtattttccagttgtgagtgtctccaaaagccaatctgggacatatgaagtaaaaagaaaacctagagagctcatctctgtattgtttcttgggtctcaaggtctctagccaaattgcattatctgcacttttcaatctttatgtttgatttatgcataatgtccagagattttagctacatttagtgtaaagaagagggaaaagtgtgtctactccatttggtccagaactggaagtactctcactgaacttccaaaagattttaatataaagaattgttggggcatttatactccaaagcctcgttgcttactttatcagtagaaagatcacatatttaggttccgaaaagtgctatgccgtttaatgtatagagcatggtcttgcttaagtgaacctagtttttaaatagtagtaaactttgacctcgagaaaggtaatttaattgctctgaactttatctcctgttcttctaaaatggggataataagttttgcatctgaacttaataaactgtctaacaaaagtctgagtagtgaacattagatatacacaatgtaaatatataagcttatataagtacttaacagctctaaaattatggagggtttggggtaagacagaaatgctaagttttaaaatgacttttcaaggatgtatggcaacacattgtccttggcgtgctggatggcaatgcttaatgcaacttagtgtgctgacttaggacctctaaaaggacattgtattaattttgaaacagaagaattacattgcaacagaggttgaaaaaaattataggtgtcaactgagaactgctctctaccagaacctaggtattaattggccaactttgctagttattcctctgaaacctgaatgaagagaaggtagtaaaggaaatcatttagtaatggaaaaaataaacacaagattttagtaggaagaaggtactaaaagccctgttaaaagagtcctgggagcttccttgactggcatttgaaattaatcttatattttcctcataagcagttgttagcatagcagaattttgatttgtttagaagtcaaatgtgatttactaattcaatccctgtggtttgagggagaaaggagtaggtccctattagaactgtgaaatcagtacagtttgctctcataaatgctcatacacaaccctcctcacttcctctttttcttgtggttctttttagtccccaaagtccagcaaccccttttttccccttgaccaatttaaaacaaaccatttgaatggaatcgtagatgattgcaatttagtgtggatttagttgcattgaaaaatgctgtcacatgttggaaaaaaaagatcaaagatcatttctcctctagaaaagcttcaggctccatattgagatgtattggggatatttcattcttcagctctcaaaatcaccctatagagttgccttcacacatatttaataacttgttgacacattgctatttatgatataaaataactgatttatctatttgatataggtatagcatatgtggccttgcttactaaagtggatgattgcagtgaggttcttcaagacaactttttaaacatgagtagatctatgacttctcaaagccgggtaaaaaatgctgatcataaccagatattattgtaatagtatcacaatcatacgtgtgtgtgtttgtgtgtgtctgtacgtgtatatgtgcttacagagtgtatttgcagggaaatgaagaatgggatcaattgcttgattaattcaaatttatatcacactttaaaactgcaatgatctgaattattgtatgttccgaagataacttattaagccattgcttttttggtttctttcttaaattgtatttaaaattggtcaaatttcaaatattaaatacaggacttacactttttaaatatactttccacaggtcatgaatgtccataaaatgctaggcattcctatttccaatattttgatggttggaaattatgcttcagatttggaactggaccccatgaaggatattctcatcctctctgcactgaggcagatgctgcgggctgcagatgattttttagaagatttgcctcttgaggaaactggtaatctggcccttttctccccctgtcatagatcactggtgccttttgaaaaatcctaagttatacatcagttattagatgactggggcccacctgcatgccctagtcctgaaagctacattaggatatatgtttcatttccactcttgtttgtttcattttcaggtgcaattgagagagcgttacagccctgcatttgagataagttgccttgattctgacatttggcccagcctgtactggtgtgccgcaatgagagtcaatctctattgacagcctgcttcagattttgcttttgttcgttttgccttctgtccttggaacagtcatatctcaagttcaaaggccaaaacctgagaagcggtgggctaagataggtcctactgcaaaccacccctccatatttccgtaccatttacaattcagtttctgtgacatctttttaaaccactggaggaaaaatgagatattctctaatttattcttctataacactctatatagagctatgtgagtactaatcacattgaataatagttataaaattattgtatagacatctgcttcttaaacagattgtgagttctttgagaaacagcgtggattttacttatctgtgtattcacagagcttagcacagtgcctggtaatgagcaagcatacttgccattacttttccttcccactctctccaacatcacattcactttaaatttttctgtatatagaaaggaaaactagcctgggcaacatgatgaaaccccatctccactgcaaaaaaaaaaaaaaaaaataagaaagaacaaaacaaaccccacaaaaattagctgggtatgatggcacgtgcctgtagtcccagttactcaggatgattgattgagccttggaggtggaggctacagtgagctgagattgtgccactgtactctagccagggagaaagagtgagatcctggctcaaaaaaaccaaataaaacaaaacaaacaaacgaaaaacagaaaggaagactgaaagagaatgaaaagctggggagaggaaataaaaataaagaaggaagagtgtttcatttatatctgaatgaaaatatgaatgactctaagtaattgaattaattaaaatgagccaacttttttttaacaatttacattttatttctatgggaaaaaataaatattcctcttctaacaaacccatgcttgattttcattaattgaattccaaatcatcctagccatgtgtccttccatttaggttactggggcaaatcagtaagaaagttcttatatttatgctccaaataattctgaagtcctcttactagctgtgaaagctagtactattaagaaagaaaacaaaattcccaaaagatagctttcacttttttttttccttaaagacttcctaattctcttctccaaattcttagtcttcttcaaaataatatgctttggttcaatagttatccacattctgacagtctaatttagttttaatcagaattatactcatcttttgggtagtcatagatattaagaaagcaagagtttcttatgtccagttatggaatatttcctaaagcaaggctgcaggtgaagttgtgctcaagtgaatgttcaggagacacaattcagtggaagaaattaagtctttaaaaaagacctaggaataggagaaccatggaaattgaggaggtaggcctacaagtagatattgggaacaaaattagagaggcaaccagaaaaagttattttaggctcaccagagttgttcttattgcacagtaacacaccaatataccaaaacagcaggtattgcagtagagaaagagtttaataattgaatggcagaaaaatgaggaaggttgaggaaacctcaaatctacctccctgctgagtctaagtttaggatttttaagagaaaggcaggtaaggtgctgaaggtctggagctgctgatttgttggggtatagggaatgaaatgaaacatacagagatgaaaactggaagtttttttttgtttgttttgttttttttttgttgttgtttttttttttttttgtttttttgctgagtcaattccttggagggggtcttcagactgactggtgtcagcagacccatgggattccaagatctggaaaactttttagatagaaacttgatgtttcttaacgttacatatattatcttatagaaataactaagggaagttagtgccttgtgaccacatctatgtgacttttaggcagtaagaaactataaggaaaggagctaacagtcatgctgtaagtagctacagggaattggcttaaagggcaagttggttagtacttagctgtgtttttattcaaagtctacattttatgtagtggttaatgtttgctgttcattaggatggtttcacagttaccatacaaatgtagaagcaacaggtccaaaaagtagggcatgattttctccatgtaatccagggagaaaacaagccatgaccattgttggttgggagactgaaggtgattgaaggttcaccatcatcctcaccaacttttgggccataattcacccaaccctttggtggagcctgaaaaaaatctgggcagaatgtaggacttctttattttgtttaaaggggtaacacagagtgcccttatgaaggagttggagatcctgcaaggaagagaaggagtgaaggagagatcaagagagagaaacaatgaggaacatttcatttgacccaacatcctttaggagcataaatgttgacactaagttatcccttttgtgctaaaatggacagtattggcaaaatgataccacaacttcttattctctggctctatattgctttggaaacacttaaacatcaaatggagttaaatacatatttgaaatttaggttaggaaatattggtgaggaggcctcaaaaagggggaaacatcttttgtctgggaggatattttccattttgtggatttccctgatctttttctaccaccctgaggggtggtgggaattatcattttgctacattttagaggtcatccaggatttttgaaactttacattctttacggttaagcaagatgtacagctcagtcaaagacactaaattcttcttagaaaaatagtgctaaggagtatagcagatgacctatatgtgtgttggctgggagaatatcatcttaaagtgagagtgatgttgtggagacagttgaaatgtcaatgctagagcctctgtggtgtgaatgggcacgttaggttgttgcattagaaagtgactgtttctgacagaaatttgtagctttgtgcaaactcacccaccatctacctcaataaaatatagagaaaagaaaaatagagcagtttgagttctatgaggtatgcaggcccagagagacataagtatgttcctttagtcttgcttcctgtgtgccacactgcccctccacaaccatagctgggggcaattgtttaaagtcattttgttcccgactagctgccttgcacattatcttcattttcctggaatttgatacagagagcaatttatagccaattgatagcttatgctgtttcaatgtaaattcgtggtaaataacttaggaactgcctcttctttttctttgaaaacctacttataactgttgctaataagaatgtgtattgttcaggacaacttgtctccatacagttgggttgtaaccctcatgcttggcccaaataaactctctacttatatcagtttttcctacacttcttccttttaggtcaacaataccaagaggggttactgtgctgggtaatgtgtaaacttgtgtcttgtttagaaagataaatttaaagactatcacattgctttttcataaaacaagacaggtctacaattaatttattttgacgcaaattgataggggggccaagtaagccccatatgcttaatgatcagctgatgaataatcatctcctagcaacataactcaatctaatgctaaggtacccacaagatggcaaggctgatcaaagtcgtcatggaatcctgcaaccaaaagccatgggaatttggaagccctcaaatcccattcctaatctgatgagtctatggaccaatttgtggaggacagtagattaaatagatctgatttttgccatcaatgtaaggaggataaaaacttgcataccaattgtacacccttgcaaaatctttctctgatgttggagaaaatgggccagtgagatcatggatatagaagtacagtcaatgttcagctgtaccctcccacaatcccacttccttcctcaacacaattcaaacaaatagactcagactgtttcaggctccaggacaggaagtgcagtgtaggcaaaattgcaaaaattgagggcacaggggtggaggtgggggggttgaataacaagctgtgctaaataattacgtgtaaatatattttttcatttttaaaaattgatttcttttgcacattccatgacaatatatgtcacatttttaaaataaatgcaaagaagcatacatccaa

SEQ ID NO: 2 - DNA, 22489 bp, Artificial Sequence
  GENOMIC SEQUENCE FOR FAM89A
cagagatgggggtgatccggaagcctggggtggggggtgagtgggttcggagctgagggtgagccagtgagctgagggtggcacagagggcgtgggggcggaactgggggtgagccgggaagctgggggttggcacagaggaggtggggacagagatgcgggtgagccgggaagctggggttcggggtggcgcgggtgagagggttcggagctaggggtgagccgggaagctgggaggtggttcagaggaggtggggacagagatgggggtgaaccgggaagctgcgggtcgcggggggcttagtaggttcggagctagggagtggcacagaagggttcgtgacggggctggaggtgagtcggggggttagagggtagtcacgcggagttggagatgaattagggcgctggaggggcgcgagggaggaggagacccgggtggaggcgagcccggctgctggacgcggacgccacccggacccggggcccgcgcaggggcctcgaggagagggggcggggccgggggggcgtggcgcgggaggggaagtgggcggggcaccgccgggaagggggcgggccgggggaaagccttggttcgctgcagcggggcaggcgcgtggccgggccgcggcgcgatgagtggggcccgggcggcgcccggggccgcgggcaacggcgcggtccgggggctgcgggtggacgggctgcccccgctgccaaagagcttgagcgggctgctgcactcggcgtcgggcggcggcgcgtctgggggctggcggcacctggagcggctgtacgcgcagaagtcgcgcatccaggacgagctgagccgcgggggcccgggcggcggcggggcccgggcggcagcgctgcccgccaagcctcccaacctggacgccgctctggcgctgctccgcaaagagatggtgagtggggctccgcgagctggggctcttcccggccgggctcgccgtcccgggaaagttcgcggggaccgcgctctgtccggaagtccccgcgcccacccgccctttcgggctcctccgccccaggcgccggcgccgtcctcccaacgacccccatttttctcgcgtgctccgtgcccacgattggaacccccgcgggagagccccgcgcgcagagggcggctttcttatgcccggcgccctcagtccggccccgctggctcggaaacctgggcgcccggaagcgctgtgcggggttcgtgcctggcctgggggcgggggcggccttgtcacctctccccgagtgaaacagaccttcccggtgggggaaaggctttcacagcggcccaacggattaacgcgattgcgttttcctaccacgaagaggacaacttttgtccgccgccagtgtagacagcagattggaacagcccggccccctttccggcgccccaggccgcgcgtccgtgatccgattaccgcgggatggccccggcgcacagatggctgcgaaagcagacgcgcaccccgggcgagggaggcggccgggtccctcagccccgcgaagctgattgcccaaaccctcttgagaaaggtgggaggtggctgtcctcccggtctgggtgctgtccatgtgagttcttcgccttgtgtctaagctccataccatgggctcagtgtttctctgtgcttgggaagtacattagctgtttgtggaccagaacacacatgatttagggtgacgctaaaagtaggacaagggcagggatttaggcaacagcgagtctttccccagctttctcggccaggcgtaggccaggcaagaagaaatcaaaaacttttcctcttttctaccatcttactggcccccatcacctcctcccaatcccctcgttttaaaagcctccctttccattcacctcgtccaggttgtctcctttccctataggtaaattgttaagaaatctaacattaggaaagctgccttttcccaaaactaaatttgccaaaaaataaattgttataggaatcttttaaatatgtatctagtgcatttaagatattgtttagaaaaattcagggtatgcatacttttttttcaggagcattatctgttctgaaaactaagacttaattgaattcagaaagcagccttaacacttttaatcaaagagatattgtcttcctactctgtagctggcattgaagtgatttccaattctcactgaaaagattttctaagcttcttacagaaccacttaaattccaagccaaccgtttttaatttattaaaaaacattcattgacataagcatcacacagctggtgaactgcattttaattagataaatctacacgtagtgtgtttacagtctgaacttggacatagcagaaccacgggggtgaagtaggaagatcatctttgattatttaaattccatacttgagcaagagatagaaaaacctcggggccgctcctgttgtgaagctgtggtttataaacatgctctggagtcttgctatggtggcttgggagtcaacgtgccattcccagaagtatttttccaggtccctcctggtgtgactgaagcacaaccacatccgtataattacgccttggaccagagctctctgtaagcctatttgaagcacaagaaaaataaacagccatctttggtctgcctggtatttagctgagataaagataagatatggctgcaggttttgacaagttcctttcaagaaatgtcacaaggcctttaaagttgcccagagaatctttcggctttttaattgatttactgacttggggccatggggtctgagtggacaactcaagctgagactccctctggggaggccttgcaaaacaagaactgggagttcattcctgagatatctgcaaaatagtttgtgttgatctgtttaaattgaaggcctgacgtcaaatctgtggcaggggacataactagatgtcatggtagaatgtgataaatgccttaaagaaatttttttttttaaagcaagcatagaaagaggggcaacttctaatagggacagggagcagggtggtgtggaagacctcagaaggcgacagaatttcgacaagggaaagaggcaccaggaaggtagctgcggagctggaactgggagtgcgccagtttgaaatgtgagcaagaagggcctgggcaggtggaccgagtggactctgagaagcctgagtagcaaggatgggcattcagcaggagaatggtattatcccagttggactttgaagaaatgaattctacagcagggtgcagaagggagagctggactttggaggctcaacaggaagatgagaggtgttcatgggagaggtgatggagtccccagcagggtagggggcttgctaatgtgaaacaagactcatgtgggagacacttttctgaagccgaagctggaggaattactgagtcaaggaagatgatgaaaaggggatcaaagataacttaagctttttcatggaaaatgtagccaagcaaaaaattaaaaattacagtgccagcacctagaaataatcacttttagtattttgggatatcttctgttaggtgcaatgtaagtgctttctatatagtatcttatttaatggtataaattctccatgagatagatactcaaagtctgttttatattaaagaattggatgctgagagttgaactcccataaggtcacagaccctaccaggtctctttggctccaaagccctatttaaccattgcagtctgctgtctgtgcacatgcatgcactctcacacacacacacatacatatatacaacacattgatcacatatattttggtttgctttttgggctgcacattgcaattattttcccagtcaagatatattataatgacttcagtgagtgtgtagtataccactgtatggcagttagcaaggttttgaagcttaataatcaatcactggtaaagtggggttcattatggcacttggggagtcaggaggagtagctgctttagggaggaaggtaatttgtcatcgcatcagctgaagagcatgttaaacatttcagaatgtggagctggaagctggaagagaggttttggtctggagatagccagtagaagagatggttggagctgagggagtaataccatctcaatgggaggagaggccattcggatgccgagggtggaggctgggagagctggagcccagggctgagaagggtctgtctcatgactgctgatgccctcctctgcttggagagttgtggtttcagctccacgtttcaacacttcctgttctagtaacccctgtgaaattctgcactactcgtaagtcctcgtcccctccccagaagggcccacttggaaagcttcaagggtcacacagatagttattgctctacagaccaaaaaagtccttttgaaaaagttgatgatgatgatttttacatcagagaatatctttagatcacgtttaagagatgattactgggtgtatgttagatagcaagtactgtggatggtttaagggtgaataggaaatatctagatgttaaggggcttatcacacctggtagatgtgggcatctttacagaaaaagaattgctttagtttagactagttttcatttttcatgaccaaagactctatattagtaatagaaacttagtttgaactagctttttcaaaaggacaatcttatagactggatgtatacagagacaggctagaactagggcttatggggaatccaggaagtccactgaggtattctcttcccctcctcctctgttttgttttttccctccattttggaacctggcctctaacagtggccaccctcaattttggccttgctgcttagttgcagtttgcaaatactgtggaaggatgccaattggcctagcttaggtggcctggccagcctgggccagccaacagtgacaaggacaagattgtattttaataagatggtgtgagcatgtggatggagtcggacactggggattctctaaagaaaggacagtttgcaaaaatggagcaaggggtaaagtagtagacatctactgcagaccccgttctatataaaaatactttgccctcaagggtcccacaatttgaaagattttttatctgctaagctgatggctagcttggctaactagatcttggttggcctttaaaatatttgcatgtggttgaaggatgtccctgactgggtgtcagctgggacccctggcacacaccagtccttgcatagatttttacatagactgcccttcccagcacccgtgcgaggttagatcatcaaccttacaggtaaccagaagtcacactagagtgtagagacacaaagaccttcagccctgggggcaggagatctttgaggagcagcatccctggggattcttgggttcagctgctcccacagtcagcagcaaggtctagtagctttgatttggaatctcttcgcctcatttttttctttaaactatcagttattttggtctcccacctgtgcagagtgggaagtcatccacacagaacttttgaattcccaaattgcaatgttgtgtaaagaattgaacctaaggaaaaaaaaagttgaatttgtgaaactagtaacaattagccttcctacattttagttgaaacaactaaatgcctaatgagcttgtccagtgaactggattccagctcattagctggaatagctgacaccccagtggagtacagtccttatcctttatgtgaaaccagtgtcttacagaggaagttttagtctttaagaggctgtgattgagtcaggctatgaagtgccatttagaataaggggattcgctcctagtgcagcattcttgattggcgttggtcagaggagactggggatgtctagcggcctttaatactgtctgttttcactagtctttccactagcatagtctagcacagcgatccccaaaggatggaccgccagctccagaatctcctaggctgcttgcccaaatgcagattttagggccacattctgtgcttctggaatcagtagctgggagaaggaatctgcctttttttttttttttttttttttgagacagagtttctatcttgttgcccaggctgcagtgcagtggcgcgatctcggctcactacaacctccacctcccgggttcaagtgattctcctgcctcagcctcctgagtagctgggattacaggcatgcgccaccatgcccggctctttttgtatttttagtagagatggggtttctccatcttggtcaggctggtctcgaacttctgacctcagatgatccgcccgcttcagcctcccagagtgctgggattacaggcgtgagccactgtgctcagcaggaatctgcatttttaacaagccgtttaagactggagaagcacatgaatcaaggatcaaaagctcgaatttggtgttaataaactatgtgatacagttctgacaagccacttcactcttttgggctaaaatctcttattgggaaaatgagaattaaatgccataaagggtccttttggccatggcagtattctttacccctcatgcctctatggttctttctgatgcctacagaagaagttggctctgtcataacttttgggcacacgtgcggggcctgtcaccaagcatattgcttggggtccccaaggacacttcacagctatacctagttgctgtgaattccttgaatgcaaagaatgggaagcagaaaaggaagaaaggtacaagtttgctattcttgagctcagttcatcaaaaattaggctgtctacaccagttattaagattttcaggccactgctaccctgtacttgtcccatccccatcccaatgtccaccctataaaagcaaaaactgaaaaaagaatatatattagtttgtgtgtatgaaagcatgcccatgtctttggtgtggggtgggggacagtaagggcagtgtgtgggtcattgcctggcttcattcacttgatgctatctccaagtgaggttagagttcttctcccgagatttgaagatataaaggattaaaagtaaaaataccactttaaactttgctctattactgtacctacctgcaaagtactataaattgatatttttcctaactcataaatatcttacaacccttctcctttttttcccttttgtttaaaggtaagcatctgttcaatgtaaatgtaaaggtgccccaataattggcagtgtgggcacctcttcatttgcagatagcctcaagtgagcaatagccctggcatttctgtaccttgcagacagcggtgcctcccctgctctgggtcctggtctcaccgacatggctgtagccccctgaggccaggtgggcaaggatgtttagggagggttcaagaagggaaccatgcctggcttgcagttcactcccaccaagctgcagatggaagtttcgcagtttcgctctgggaatgcctgcaggaactccatggagactttagaccccactttgaaaaaccaagcttttcataatgctgtggaggaaaccagacagaccacagactccatgctcaggaagcgatcccccgaggctggctgctcagatatttgcccccgttgccagtgtcattctccatatggagccctggcctcctggccgccttggcctttgcccacgtgttcctaatgtttggaagtgatgattagacaggagtcataaaggctgctcactacttcctgtggctcgttccccacagacacttaacacagatggtcaccctctcccaggaactctggagacagaaaaacctttagcctactttagaagtctacagaaattcattaagacatgtggcctttcccgtttttgtgggcactctctgttcacttccttgattggccccgacagccatgagctggcctagttttgcaggtgtgcgctttctgagtctcaaggattcgggagggaggcaccatctttgaccagtggagggatctggggagaagggagggcctctgtcctctgcccagagctccctagtcagcgggtaattgttggggaaccccaggcctgtcccagccaggagagcctaggctgaggaagaaggtgactgagatgcaggtgaaagcgagtgtattcttaggtgggtgatttggttaacctaaatggattaataaagtttctcagctttaatttctaataaggtaaatattgacaggtatagctcacataaacaaaagctctttgggactctcaattgcaattaaaattggatataaaatatccaaattaaatgctgctaaaagagaagtggcaaggtgtttaacattccttataaccacggatgtatacattaagacaataaggtatcatgttgtacctccaagactgacaaaggtagaaaagcatgatcctgtcacagtgagggtttggagaagtaaaccttctcatgcattgctgggggtggggggtgggggctggcgggggcggggtggggtggggcggtgtaaagtgctgcagggttttttgagcgcagtttggtaatacctctgaaattgaatatgtgcctgtcttttgaccttgtaattgcattttttaaaaactctgaaatggctttctattaaatagcaaagcagaattgcaatataattttaaaatatgtttaagttaggtcacaaaagggatgtaaaatgtttgcagtatgactgttaaatcttcatacagctaaagccaattattgactctttcttataccaatacagacataaaattattttgtgatgaaaagtagtccaaattgaatcactttattggtaaacgtctttcttcccattacattttcccattgctttggacttgaggcccggggttggggaggattggaaaggcgccttgggcattcttctctccttgtcctccttgtcccccacaatttcatattcacaagtgtaccttacagaagcatccacacaagtggataatggcacttatacatggatgtgtattgcaggattttttataatagtgatagaatactgtacaattgttgaaaagaatatggtaactatatatgtatatagaaagatgttcacagtgtaaagttacaaaacagtacttacctaactttgtgtatgtggtaacagtagagaaaaaacaatatgagtgtgcatagtgctttgaggaatatatgctaaactactacaagtggatatctgaagaaccacagtttcaaagtgtggtctggggacctctaggggcccctgagattctttcagagggtccataattatatgatggtgatattgacaaatgtgactttttggttattatataagaaaatgtaccaacatttggaagatcctgcataatttattgaatcaattttccacttttttcatatgactgtgcttgatattaaaagatccattcaaagtgcaagactgatgggttttaatgtaatagagtgtgaacatttcattggtatagttccaaattccacactaaacagcagtcaactaaagggcggtagcaaagaggaatatccacaattgtctgaaaaggctattgaaatactccttcatttcccagttatacagctgtatgaggccagattttcttcatttacttcaaccaaaacagcacgtcacaaaggaccaaatgcagaaccagataagccagatatttaaaaagatttatgaaaatgttatttgtgttagcatgtaataggtttattattattattattattattattgagacagagtctcactctgttgcccaggctggagtgcaatggcaagatcttggctcactgtggtctctgcctcccagggtcaggtgatcctcccacctcagccacccaagtagctggggccacaggcaaatgccaccacacccagctgatttttatattttttgtggagatagagttttgccatgttgtccaggctggtctcgaactctcaggctcaagtgctccacctgtcttgtcctcccacagtgctggaattacaggtgtaagtcacctcacctggttggtgacttttaaattttctcagttttaatttctagtaatgtaaatattgataggtataacccacataaaccaaagctctttgggaccttcaataattttttagagtgtttggagaccaaaacatttgaagtctgctattttataacagggaattaaggagaactggtttgtatgattacgaaccatttgaatttataatacaattagagtgtttatttttataatcagaaaaaaaataaaagaatgtacaaagacatttcttaaagaaaatggtcaattgcttttcttcatctatatccaggacagaacaagaggaaatgggcttagtttgtatgaatgttagtttaggttagagataaacaagaatgtccttctgagaattgttaaattgcagaacagtctctgtgtcagtgtggatgccctcacttgtaagttagcagaaaatccaattcaaacagctttacctggtagaggagtttcctggaaagtatagaggtgggatgtgctttgggtttaatgggggttaatctgggggcacagtcatgcaacccggtttatcttctgtctctgaatcctgatggcgctttagagtctagtcctcagcttggcaggtctaaaatattaacaggagatgaagctgaccagatgacacgaatatgtttccgcccatgggaggagaaggctacataggagaccaggtcatcagaagccgtttagtgagcacagagctggaacccaccagggagctgagagtccttcaagggtgtttctgtcaagcttgggtagctgggctcatagcccgtctccaactgcatcaacactgatgaagtctctcttcggctttttctaaacactatgcagggcagcatccttcagtcaacatatcttttatcagaaatcaggttataatcgattggatctctgctttcttcaattacagtccaggcctgtggatataaactagacactgtgattagatttggggcatttaccaagtctttaaaataaatttgtgagccatctgtatatacttactcattcattgtgtttttaaaagataactgtgaaagttttctcattgttaatacattttcacaatagaaaacttagaaaattcagaaaagccaggaataaaaatggcctgtgatccaagcaggttgctataccactgctgagactggggcctctctcttcatcttccctgtacaggcagtgcagggtgattgtcaaagcacccatttcagagtcctgcagatctggtcacctccccactctgccactgactagatggccttaggcaagggcctttgtcattctttttttttttcttttttttgagacagggtcttgctctgttgcccagattggagtgcagtggtgcgatcacagcgcactgcagcctcaacctcctgggctcaagtgaacctcccacctcagcctcccaagtagctgggaccacaggcacgtaccaccacacccagccaatttttaaaatatttttgtagaaatgagggtctcgtcatcttgcccaggctggcctggaactcctgggctcaagcagatcctcctgcctcagcctcccaaagtgctgggattacaggcgtgagcctgtaatctgcaaatggcagttttttaatttctaaaaaaatcttaacatttttcatgatgttttggtttaaatcaacacaaatttccttttaaaggttcctctcatcttttaagccttgtttcctagtggtcatatttctattgtccttgctttaagttaggaagaactctctcccccatgcagcctccagagatactcagagactttcagtgacttaacacccagctgggagccaccgccctgtctggagtgtatttgtatgtggagcctactgttttgaaaatcccaagtgaaaggaagcagtttcaagggtggtttgggcttgtttggccccattgttgggaatgctgtggctctcggggccacctgtgtgtgttgcgggaggggtggaggggagctctgggcatgggagaagaggagtgaatgatcaggaaggaagcaggaagcctgagcagagagcggaaggacctgcgctcgcagtttacggccatggaagctgctgattgttcttgaatttaaagtggagaataagggaccacaaattgcagggtttgagcattccatgtttttcttaaatgagcctgtctgcattttcaaaacgtgtgctttcaaaagagagctgtattttctgaatccagctgtgaatgtggagaccagccgtcctccaagggcatgcgagaacacaccgttgagatccaggctgcttctgctcggagagtggcttgctcggcggctccccagccactctttttctggaagggtgagaagttcttgttcatggtgacttaaccatgtcttgcaatcaagtccttttggatggttgctctctccccttcctgcatccaagacccacataccttcagtgtagagagactgaccaccagatctgccctctaaagagcgctcctggaggaaacttggttgggtgtctttggcccttgatgtgatgggaggcacgcggggactcagtggtctgatgcttcccacagggacaccttgtgtacagggcactcggcggctgcccgttcagtctgcacctctgtgactgcccgagggatgcagccagagggtctgtgggtgccagcaccaccccactgccaggccacttctgcggctacgtgttctctgggagggtgagatctctgcagccaggcgttttcactgattcaccaaatatctgcctgtctgctctgagtttctgggctgggtgctgagagatccaaaagggaaatggtgtttgccttcatggagcttgtcctgtgtcaggagagagaagacctgtgtgcacaccgataatatagagagtagtaaatgtcctaagacaggtggagacgccgagggcaaaggatgaacactggctgaaccaatcacagtctgaagagtggagggaatcaggtacagggcgggtggtcgaggagcattcacagatgcagtggggatgagggtgtcatgggggacagtcggggctgtgcaggttgggagtcaagggcgtaagcctgaagaacagtcagaccagatggtggagtgctgcctacggatcttccacctccctctagaaaatgttaagtgtcgctgtttaaacagccacagctgaggaagaggggcccgggctaggaagtctggtttactgtgcagtgacttaccttatgtcctccgagctgatttagaggatttctggtaaatcaggaagtttagtctggtgcctgaagacagtggcattgagaggctgggaggtgtgtaggcgtgtgtgtgcgtgtgcatatgtatgtgtgtgcgtctaatccttgttaaatccgtctgaacttttgccatgtgtcgggttgtgtaataggtgtgtgcggggctgcgctgtattcctaggcggtcaggattcctttctaggccagtgttccacctgacgacaaggcagctttgtgagtcatctgggtgctacagtgcagaagtgtccagggagagatcctctttgctttcgactccctgccgggtgcatcacctcggtgggcctgggaataccttggaaatggcactgtcaggagaaaagcctggagccacgtgtctggctggaatggggtcatggggagtcagagcctttgaaacctagaagcgttcaggctcctgtgtttacctgggccgacctcaaaccatcccaggaaggagaaaagcagacctgctctgataccagggtgcccactgctacttaggtgtttttccattattcattcctggggtaagaaatcgagtcttgggtttacccaccctactggtgtcagagggactcagcaggagagtagatctaggattccagatgatcttcttccatggtttttgagcacatactatgtgaccccgagagagtgtggctttctcgattaaagttattatttcttttatgaaatcctagcaaagatagggacgtcagagctggccgagtcagactcctgggggcatgttgatggcatccagatgcaattctgcagaggaatcctggaaaacaggagtaagtctagaggaaaggccacgggtgttagtggacgagaggtcataatgaaaataggggaagggcctgagatatttagcttggagagaagaacacaggtttggtttttgttttagggcatggggtggtggaaagtaaatgaccttcagattaaagggtagtagttaggagagagttaaattagatctgtttggatgctcagctgtcacacccagcatcaagggctctgtggggcctccaggctgggaggctttgactttgtataaaataatcgtattggtttggagaggagtgcagtggtttggaaggtcctccttttggggtttgaggtaagatatcccaagtcttttcctatttgagagtttcccttcctcatgaggcagtgtcactggcacgttgtcaccctgcctgactatgctggctgtcttctgagcgaaggtgaccatctggttccttctcatgtaccacctcagtgctggattgggagaggagcgggaggaacacagtgggatggggcgcttctgttttcagagcctggctgtacctgctgctccttcctgaggtgagtctgcccactagcagagtggaaaagaaaccatggaaatactaacaatgagaatagaggctattgattttttttttttttttttaggagctgagcaatttatccacagtttctcagctggtgagtggcggagccaagatctgaacccaggcagggaggtaggcaggttccagagcctgcacttttaattctgtgctcttctgcttggctggcctgaaattccaggcttacaggataataaatataagtggcccaggaaaatcagaaagatatttgtgtcaagatcactggttctttgctggaactgagcatcagcatcatctgggtactttttgtattatttatttattttttcaatagaaaattcctaaactgactgacttttctttccctccttctctcccttccttcctttcttccttctttctttccctgtctctcctttttttaatagaaaattcccaaactatggataatttttaaaacacaaatgccagatatgctgtttccctccctcttgacagacacacatcctttcgaactctaatcaagaaaaagagcaagcagtggtgtctgccttagggtgtggtggcctgggcatctcttaagttgcccattgcttgcctattcaaggtatgcttttgagatgccattgaataaagtttgctcctgagtacagtactggaaactgtctgtctttcgcttgcagttcatttaggacagagaagcaacagtttatatagggtcacaaagtgtttgagctaaccatagatgagcgagcccaaatcccccattttataggctggcagagggtcgggacctcaaccaagccacagaggacggcaaagctgggcctggagaccacgctcccgacctgcagctgaggtctcttcctaagaaagtttagaaattctggtgtcaagggtagttgtggtggccgggcacggtggctcacgcctgtaatcccagcactctgggaggccgaggcgggtggatcacaaggtcagaagatcaagaccatcctggctaacacggtgaaaccccgtctctactaaaaatacaaaaaattagccggacgtagtggcgagcgcctgtagtcccagctactcgggaggctgaggcaggagaatggggtgaacccaggaggcagagcttgcagtgagccgagattacaccactacactccagcctgggcaacagagcaagactctgtctcaaaaaaaaaaaaaaaaaaaaaaaaaagagtagttgtggtagcaacagaacccacctctctatctggaagtcttcttgagtgtcttagcaaaagatgctctgtaggctgggcacagtggctcacacctgtaataccagcactttgggaggccaaggcaaatcacttgagcccaggagtttgagaccagcctgggcaagatggcaaggccccatctctacaaagaatttctttaaaaaattagccaggcatggtggtatgcacctgtagtcccagcagcatgggaggttgaggcaggaggatcccttgagcccaggagcttgaggtggcagtgagctatgatcataccaccacactcctgcctgggtgacaaagcaagactccatctctaaatgtgtgtgtgtgtgtgtgtgtgtgtgtgtgcatgcaatgtaataaaacatagttctgatttttatggtctattcaggccatagtagagagacagccagtgttcacttggcaatttagaaaagttggagggtatgaagagtaaacctggaatttaacacccaatctatttacaagatgatcactttttaccaggcctcagcttccttttgtgaaagccatactatcttatgtggaaaatcttattgctaggtaaacgagtcatttcggtaattataaaatctgtaaatcctctgacactttctgtgtgcttttctacatgcgcgtacccatgcatctttttttttttttggttcaaattaatggttttatttccatctttaacactagcagaggagtccaaagcagactgatatccatggatgtagtttaaatgtaacaaagaaagagttgaactatgtacattgaaaaaaggaaagacattttttcataccaacctttccctagtttgcagtttctgaatagtagaaacaaaacacatttttaaatctttttatcaatttaatttaggacgaagtacacaacttttataattaaccactgaagttgtcttcaaggataaaacttaaagaaattttaaaatgggtgttaccatattttattagtggactgactccaaggttgccttgctccaagtctgggcattgtgacattcccgtgatgcccagaagaaagttaatggcaatgatgtccagtcagggggcagacacgctacacatcacaatgatgggagctgaggattctgccctcttcaactccaagtagaaaattattattttcattcaaactaactggaagtgagccaaacagttaaaaagtcagaatgaagaataaaacaattttcttttcacatagaggagggacactccttcagccccgtctaaagtgaattctgtgctgagtcccttctccttcagaagggtaaactgaaggtcagttattgctaacaaagccagaagtggcccctttcccaccctgaagatgtttcacacgaaaaggctgtttgttttgcttgaagccctctgaggaaggagggcagcggaagaggaggcatgccggcactgtaaggcctctctcgttagccaccgccaggccctgtgctgtcaggggcagcttgggccactttgctgcccctgagcgaacctgaggctcccacctacctgtggagtgaaggagaggttgtcctctgggcccctgtttcaccagtcataacctatggagcagtcaaaggcccaaagcatccaagcccagtgggcttctgaaataaacggcacggggttgggaaggatgagaaagccaagtcaggtgggccaggttctccgaacatggggcaacagtgacctgggcaaaaggctggaactgagcggctgataaggccacaattactgccaccacctctcagtatctacacggggggcagatgttaggcagtgggaactgaggactggagggcgtgtggcaaacaccggatggattttatcagaaaagagaggacacccaaacatgtgcctgtcctatttatcttgcatgtcctgtgccaggtgaaggacgctggagcatgggtaaggttcctgagaacaactggtgggcagaaatgggctgggatgggcactgctccacaggcaacattaagcctctgagggggacactaatagtgctacatctggtgggctgctgaaaagtaggtaacgaatggcctttattgcactttttcattcttaggaaacgggattgccctgcagagcttctcttgatttgcagaaatcactgcagatcaatgataaggtgcaggcagaatcacgggtgacctctgactctcaagggaagaagtccagtgattggtcttttcagggcctcaaggggccactcttgcacctgggatcctcgagctgggtgaaccgggtctggcttggtcaatgtgtggcaggcagattggtcgaccggcagacacttgggacaaaaggtggtgtgcccgggaaagctggggcaaactttccaaacggaaaatttcttggcaaatgtgcaggttctgcaaccagactggaaccacgattcccagtgtgcctgactccctttctctcactctagaactggaccaccccagaggaacagagatggcctgggagggccctgggtccagcgccatagcatcaaactggagataacaaaaggaaggggttggaaacaaaagagcagtttacatatcagacgtgggtttcaaaacagtctttttgagctcaggaaaatggaggcagataccactggagaacctgattgtccatccgtctctcctgggcgtctctgaatacttcatatatgaatggagtggtactgtttgtggttgatctttttcctacaagttgggcaagtattagcgttcttcagggaatcacggaggcactggctacagaagacatggccacattctgtggaaacgatgagacgtctattctgcacgatctctgaatatctgtccatgcagataggacaaccgacagtacccgagggcctgaggcctatagcgccctcatccctggtgtttctggaagtgtgggtagtcacatacacgtctctgtccctggacaacaactcatcgtcactgctcaccatgcagctgtcagcatggtcctggggcagcctcctagcattcctccttggtcttcttcttttgtcaacaatcacaacagagtcattgtgagtcagatcaaccaccacaggctctaaagattcacaagtgaggtcaacaatttcatctccagcagtttccacgagttctatgggttctgcttccaaggaaatctcaggggtggaggttgcttcccgtgttcgcttctgggcttgtctagaatttattgctccacctcgacgctttcttgtactcattgtgctctttggtgcctttcgtttcctaacagaaaaggaagtgatctataccaaggtttgcagggaagtcgaatgttctcaacctttcgtgccctctggttaatcatctggcttgcaaaagaatttggatcgggacagatttccagtattttaaagtcctggagctagttaggtctgcaggcgctgccaccggcgcactccagagaagaagctccttctccagccgcccaggagagctgtacccatgcatctttagtgctttagcccgggaggcattagaatcctgtttattgagtggattgatattgaattgccctaatagctccataagagaaattattgttccattttgccatcaaccaaggcacggagatgaaggtgataaataccttgctcaggggccaagaagccgaaggcaggtcccctggtgtcttcttgagtttcttcccgttgccattcagagcagggtctgtggaacagcagcatagcacggaatcaccataggggcttggtggaagcacagccatccagtggccccagacccactgaatcagagtctgcttgttgaacaagatccccgggtggttctcatgcactttaaaggttaagaggcaccgatgctggtctatgctgcatttccaagaggcttaactgttctctctttggtattggtgtaaacgatgcatttcctgttctgactgtgaccgtgctcttttctctgggatgggtggtgggggagggaggaactggaagataaacaagtatatgacttttataaatgttctgtgttcttttgctgcttgtttttgtggggctagttttcaggaggaactgtagagcccttcatcttccagggcttcctcatattcagtcagttactctggggagggatcccagaaccatctgggataagactgaccctgcctggaggagagggaggcagtgtaacctctgaccactgaactgcacagaggtgggtgctccagggggatgtcacgttggccagctgctgtcactggcaaagggcattctgttgcccctgggagttgagaatgactgcatcagtcagatcctaacgcagtagcagggaaggccaatgtgggtcttctccgagtctgattgggagaggaagtgacacactcgtttcttggcgtccaaagtgaaagcaggtggggccactagaatatgcagtgctgttgcttcatcaggcacactcaggagcgccagggtaaattctgcaggctgccctggttgccccacagatgcgatcctcactggactcaatgagtaacgtctgaggtatgggcataacacaattaaggtgttctcaaaactggaaatccaaagcatccgagtgatgctctgaatcatgcgccgtgtggaaggaatgtgctggcaggcgcagatcgccggctgagtgttccactgaaattaaactcaagtgctgacttctcgttttttacctccccaccccttccctcaaggttggtctccgccagctggacatgtccttgctctgccaactgtacagcctctacgagtcgattcaggagtacaagggggcatgccaggcagcctccagcccagactgcacttacgctctggagaacggcttcttcgatgaagaggaggaatatttccaggagcagaactccctgcacgacaggagggaccgaggccctcctcgggacttgtcactgcctgtctcctccctctccagcagcgactggattctggagtccatctagagggtcttgggagggatgtgactgttgggaagcccttcctactggacacgctgtcatcatttgctgcttctcttgcaagaaagcacctccgttgtggacggtcctcgggcacaggggatgagcgctaccagtttcatttgtaggcagggagttctccgcggatgcatggtggcagtctgctttgatggcagcagtttctgcttaggtgacctagaggtcctcagcagtatcctccacacctatttattgaggtgcacctgctggggattcataatgagaatataacaagaggatctcggtgaaaggccttagtgggtgttttgtgtgaggtggcttgtagctagctacttccttacagatggtagagtattccaatcctctttgtgttagggttcttgcttccagtttgggatgtattaaaaccaccatttcactgcttcccttcctcaatatgctctgcagcttttcttgctgtttaaacctctcgcctcagctttatttatttgtaagctgcattactaactgcccagtgattcggtgaaagctttttactgaaaaagttaacatttctagtcatcccaatcaactggcttttttcaaccaaaattttatatcattctttgtctatcagatacgagaggaaggaagataatacgaagacatgttgaatagtgaaaaaaaaaaaaagaacacaaaaactggggcaagccaatgtgatgtatcactcactgtaagatggcaaatgttttcatttttaagattccgaatgtaaactagtgtgctagaaagcaaaccacccgccactcaaaccagtaattaccttaagccttaatatatttattaaaatactttatgagaacattacactttgtaggttaaaaatgaggataaaatgctaaactatctgtgtcatgtgttattttattctgaatttggaatcatcaactttcatgacttgaatgcattgagtccagtcaaataatgaaagaaaattagtttgtttttctgccactaaatgcatttgaaacaagattgactctgttgagcttaaggaatcgttttagcaagagtagatcaccatttacagctggttctcagtgctcttttttttctttgagacggagtctagctctgctgcctaggctggagtgcagtggcacgatcttggctccctgcaacctctgcctctctgggtttaagcaattctcccacctcagccttccgagtagctgggattacaggcgcctgccaccacgcccagctgatttttgtatttttaatggagatggggtttcactgtgttgtcctagctggtcttgaactcctgacctcgtgatccacccgcctcggcctcccaaagtgctgggattacaagtgtgagccaccatgcctggctgctcttctgtctttgaatgctgcagactccttcatctttcttttggtgtgataattgctcactagagcgtccttcaggttagggagaggaaggcacctcaatgtcatgc

SEQ ID NO: 3 - DNA, 50 bp, Artificial Sequence
  IFI27 probe
ccaagttcatcctgggctccattgggtctgccattgcggctgtcattgcg

SEQ ID NO: 4 - DNA, 50 bp, Artificial Sequence
  IFI44L probe
gtgggctaagataggtcctactgcaaaccacccctccatatttccgtacc

SEQ ID NO: 5 - DNA, 50 bp, Artificial Sequence
  IFIT1 probe
tgaatgaagccctggagtactatgagcgggccctgagactggctgctgac

SEQ ID NO: 6 - DNA, 50 bp, Artificial Sequence
  RSAD2 probe
cgctggaaccttgggcaaggaagaatgtgagcaagagtagagagagtgcc

SEQ ID NO: 7 - DNA, 50 bp, Artificial Sequence
  IFIT3 probe
aaaacaaaatcaaccgggaccccagcttttcagaactgcagggaaacagc

SEQ ID NO: 8 - DNA, 50 bp, Artificial Sequence
  IFIT3 probe
acaaatcagcctggtcaccagcttttcggaacagcagagacacagagggc

SEQ ID NO: 9 - DNA, 50 bp, Artificial Sequence
  OTOF probe
gcccgtcaagtgctgcccctgcctgtgtctgggtttctgttggctgtttt

SEQ ID NO: 10 - DNA, 50 bp, Artificial Sequence
  IFIT2 probe
gctgacccagcatcagccacactctgggttggaaaatgtttgcctgttgg

SEQ ID NO: 11 - DNA, 50 bp, Artificial Sequence
  EPSTI1 probe
gggagtcacttgatgctttcaggttaatcagagctatgggtgctacaggc

SEQ ID NO: 12 - DNA, 50 bp, Artificial Sequence
  SERPING1 probe
tgggaccagcagcacaagttccctgtcttcatggggcgagtatatgaccc

SEQ ID NO: 13 - DNA, 50 bp, Artificial Sequence
  OAS1 probe
agagagacttcctgaagcagcgccccaccaagctcaagagcctcatccgc

SEQ ID NO: 14 - DNA, 50 bp, Artificial Sequence
  IFI6 probe
tgcgccgacgatgcccagaatccagaactttgtctatcactctccccaac

SEQ ID NO: 15 - DNA, 50 bp, Artificial Sequence
  HLA-DRB6 probe
aaccccacagccttgatggcagcgcctcgtcttcaacttttgtgcttcct

SEQ ID NO: 16 - DNA, 50 bp, Artificial Sequence
  HBZ probe
gtcctggaggttccccagccccacttaccgcgtaatgcgccaataaacca

SEQ ID NO: 17 - DNA, 50 bp, Artificial Sequence
  HS.386275 probe
tgttcttccccatgtcctggatgccactggaagtgcacactgcttgtatg

SEQ ID NO: 18 - DNA, 50 bp, Artificial Sequence
  EIF2AK2 probe
cgttctctgcctcacatagcttacaagccagctggagaaatatggtactc

SEQ ID NO: 19 - DNA, 50 bp, Artificial Sequence
  IFIT1L probe
aggccttgtggcaccagacataagaccccctgaaagtatcatccctcctg

SEQ ID NO: 20 - DNA, 50 bp, Artificial Sequence
  FCER1A probe
gaaccaggaaaggcttcagacttctgaacccacatcctaagccaaacccc

SEQ ID NO: 21 - DNA, 50 bp, Artificial Sequence
  C21ORF7 probe
gtgacctcacagtaaacatctctgcctttgcctgtgtgtgttctggggga

SEQ ID NO: 22 - DNA, 50 bp, Artificial Sequence
  GYPE probe
aggatgtggcctgcatgctgcctgatcttgcctagaaccagctgcacctg

SEQ ID NO: 23 - DNA, 50 bp, Artificial Sequence
  GYPB probe
tggagaaacgggacaacttgtccatcgtttcactgtaccagctcctgtag

SEQ ID NO: 24 - DNA, 50 bp, Artificial Sequence
  HBM probe
tcgtgctgcgcgtggacccagccaactttccgctgctaatccagtgtttc

SEQ ID NO: 25 - DNA, 50 bp, Artificial Sequence
  EIF1AY probe
ctgaggatggttctacagttgggattttggccatcatcaaccaagaagag

SEQ ID NO: 26 - DNA, 50 bp, Artificial Sequence
  LOC649143 probe
ggttggtgagagcttcacagtgcagaggcgagtccatcctgaggtgactg

SEQ ID NO: 27 - DNA, 50 bp, Artificial Sequence
  HBD probe
ggctaatgccctggctcacaagtaccattgagatcctggactgtttcctg

SEQ ID NO: 28 - DNA, 50 bp, Artificial Sequence
  FBXO7 probe
aggcgacgggaagcgcgggtggtcggctggggtccggctcctggagaaca

SEQ ID NO: 29 - DNA, 50 bp, Artificial Sequence
  KCNMA1 probe
ggttctgcatgacctagccactgctgggggttttcttctataacgttgtc

SEQ ID NO: 30 - DNA, 50 bp, Artificial Sequence
  MERTK probe
cttccttaccaagtgaactccatggccccaaagcaccagatgaatgttgt

SEQ ID NO: 31 - DNA, 50 bp, Artificial Sequence
  EBI3 probe
gagctgccgggcaacctcagatgaccgacttttccctttgagcctcagtt

SEQ ID NO: 32 - DNA, 50 bp, Artificial Sequence
  FAM89A probe
caggggatgagcgctaccagtttcatttgtaggcagggagttctccgcgg

SEQ ID NO: 33 - DNA, 50 bp, Artificial Sequence
  UPB1 probe
gaaattctgcctgaggacagcagcccagtgcttggcgagagttcctgaca

SEQ ID NO: 34 - DNA, 50 bp, Artificial Sequence
  FAM89A probe
gatctcggtgaaaggccttagtgggtgttttgtgtgaggtggcttgtagc

SEQ ID NO: 35 - DNA, 50 bp, Artificial Sequence
  EMR1 probe
tctcagcttaacatggaaatgaggatcccaccagccccagaaccctctgg

SEQ ID NO: 36 - DNA, 50 bp, Artificial Sequence
  PTPN20 probe
gcatcctgaggtggccaagggcagtggtgctccagatgtttctgtttctg

SEQ ID NO: 37 - DNA, 50 bp, Artificial Sequence
  TMEM119 probe
gtctggcagcctgtgtccacaatattcgtcagtcctcgacagggagcctg

SEQ ID NO: 38 - DNA, 50 bp, Artificial Sequence
  SLPI probe
ggatcctgttgacaccccaaacccaacaaggaggaagcctgggaagtgcc

SEQ ID NO: 39 - DNA, 50 bp, Artificial Sequence
  S100P probe
aatgatgccctggagatgtcacagattcctggcagagccatggtcccagg

SEQ ID NO: 40 - DNA, 50 bp, Artificial Sequence
  PI3 probe
ctgactgcccaggaatcaagaagtgctgtgaaggctcttgcgggatggcc